European Patent Specification EP 3 795 582 B1, published September 13, 2023. Title: Compositions and Mehtods for Controlling Plant Pests. Applicant: Syngenta Participations AG Bramlett, Matthew Richard Seguin, Katherine Kramer, Vance Cary Rose, Mark Scott. The sequence listing filed with the application follows.

SEQUENCE LISTING (31 sequences)

SEQ ID NO: 1 - DNA, 3507 bp, Bacillus thuringiensis
atgaatcgaaataatcaaaatgaatatgaagttattgatgccccacattgtgggtgtccggcagatgatgttgtaaaatatcctttgacagatgatccgaatgctggattgcaaaatatgaactataaggaatatttacaaacgtatggtggagactatacagatcctcttattaatcctaacttatctgttagtggaaaagatgtaatacaagttggaattaatattgtagggagattactaagcttttttggattccccttttctagtcaatgggttactgtatatacctatcttttaaacagcttgtggccggatgacgagaattctgtatgggacgcttttatggagagagtagaagaacttattgatcaaaaaatctcagaagcagtaaagggtagggcattggatgacctaactggattacaatataattataatttatatgtagaagcattagatgagtggctgaatagaccaaatggcgcaagggcatccttagtttctcagcgatttaacattttagatagcctatttacacaatttatgccaagctttggctctggtcctggaagtcaaaattatgcaactatattacttccagtatatgcacaagcagcaaaccttcatttgttattattaaaagatgcagacatttatggagctagatgggggctgaatcaaactcaaatagatcaattccattctcgtcaacaaagccttactcagacttatacaaatcattgtgttactgcgtataatgatggattagcggaattaagaggcacaagcgttgcgagttggctcaaatatcatcaataccgtagggaaatgacagtaacggcaatggatttagtggcattattcccatactataatgttagacaatatccaaatggggcaaatccacaacttacacgtgaggtatatacagatccaatcgtatttaatccgcctgagcgtccaagtggcgctttctgcgaaagtttttatactatccgagcggctcgagaacgtttaactttttcgcaacttgaacatgcaataattcgtccgccgcgcttgtttgaaaggtttcaagctttagggatttatacaggcgaggcgcgactgaatgcaaatagtgctccaatgaactattggattggacattttataagaaatacacgtttaggtgactcaacaacaattactacaaattatggaacaaccaataatcgtttaactaacttcagtatgccttctgatgtttatcaaatcaattcaacctcaagtaatttagccgctattttaggcactttatatggggttactagagcacaattccattttggatcaggaagtttttcgacgtatgtcggacaaaatagcgttcttccacaatgtcatcaaaactataattcaatagaagaattaccaaaccaaagcgatgaacctacagttagaagttatagccatagattatctcatatcacctcttttaatttcaatgtacagcttaataatcctttaatttctgcgggcaatatgcctgtatatgtgtggacacatcgcagtgtggaccttactaacaggatttcttcagatagaattactcaaataccagtggtaaaggcatatgagctaagtagtggtgctactgtcgtgaaaggtccaggattcacaggaggagatgtaatccgaagaacaaatactggtggattcggagcaataagggtgtcggtcactggaccgctaacacaacgatatcgcataaggttccgttatgcttcgacaatagattttgatttctttgtaacacgtggaggaactactataaataattttagatttacacgtacaatgaacaggggacaggaatcaagatatgaatcctatcgtactgtagagtttacaactccttttaactttacacaaagtcaagatataattcgaacatctatccagggacttagtggaaatggggaagtataccttgatagaattgaaatcatccctgtaaatccaacacgagaagcggaagaggatttagaagcggcgaagaaagcggtggcgagcttgtttacacgcacaagggacggattacaagtaaatgtgaaagattatcaagtcgatcaagcggcaaatttagtgtcatgcttatcagatgaacaatatgggtatgacaaaaagatgttattggaagcggtacgcgcggcaaaacgcctcagccgagaacgtaacttacttcaggacccagattttaatacaatcaatagtacagaagaaaatggatggaaagcaagtaacggcgttactattagtgagggcggtccattctataaaggccgtgcacttcagctagcaagtgcacgagaaaattatccaacatacatttatcaaaaagtagatgcatcggagttaaaaccttatacacgatatagactagatgggttcgtgaagagtagtcaagatttagaaattgatctcattcaccatcataaagtccatcttgtgaaaaatgtaccagataatttagtatctgatacttacccagatgattcttgtagtggaatcaatcgatgtcaggaacaacagatggtaaatgcgcaactggaaacagagcatcatcatccgatggattgctgtgaagcagctcaaacacatgagttttcttcctatattgatacaggggatttaaattcgactgtagaccagggaatctgggtgatctttaaagttcgaacaaccgatggttatgcgacgttaggaaatcttgaattggtagaggtcggaccgttattgggtgaacctctagaacgtgaacaaagagaaaatgcgaaatggaatgcagagttaggaagaaaacgtgcagaaacagatcgcgtgtatcaagatgccaaacaatccatcaatcatttatttgtggattatcaagatcaacaattaaatccagaaatagggatggcagatattatggacgctcaaaatcttgtcgcatcaatttcagatgtatatagcgatgccgtactgcaaatccctggaattaactatgagatttacacagagctgtccaatcgcttacaacaagcatcgtatctgtatacgtctcgaaatgcggtgcaaaatggggactttaacaacgggctagatagctggaatgcaacagcgggtgcatcggtacaacaggatggcaatacgcatttcttagttctttctcattgggatgcacaagtttctcaacaatttagagtgcagccgaattgtaaatatgtattacgtgtaacagcagagaaagtaggcggcggagacggatacgtgactatccgggatgatgctcatcatacagaaacgcttacatttaatgcatgtgattatgatataaatggcacgtacgtgactgataatacgtatctaacaaaagaagtggtattctattcacatacagatcacatgtgggtagaggtaagtgaaacagaaggtgcatttcatatagatagtattgaattcgttgaaacagaaaagtaa

SEQ ID NO: 2 - DNA, 3471 bp, Bacillus thuringiensis
atgaatcaaaataaacacggaattattggcgcttccaattgtggttgtgcatctgatgatgttgcgaaatatcctttagccaacaatccatattcatctgctttaaatttaaattcttgtcaaaatagtagtattctcaactggattaacataataggcgatgcagcaaaagaagcagtatctattgggacaaccatagtctctcttatcacagcaccttctcttactggattaatttcaatagtatatgaccttataggtaaagtactaggaggtagtagtggacaatccatatcagatttgtctatatgtgacttattatctattattgatttacgggtaagtcagagtgtcttaaatgatgggattgcagattttaatggttctgtactcttatacaggaactatttagaggctctggatagctggaataagaatcctaattctgcttctgctgaagaactccgtactcgttttagaatcgccgactcagaatttgatagaattttaacccgagggtctttaacgaatggtggctcgttagctagacaaaatgcccaaatattattattaccttcttttgcgagcgctgcatttttccatttattactactaagggatgctactagatatggcactaattgggggctatacaatgctacaccttttataaattatcaatcaaaactagtagagcttattgaactatatactgattattgcgtacattggtataatcgaggtttcaacgaactaagacaacgaggcactagtgctacagcttggttagaatttcatagatatcgtagagagatgacattgatggtattagatatagtagcatcattttcaagtcttgatattactaattacccaatagaaacagattttcagttgagtagggtcatttatacagatccaattggttttgtacatcgtagtagtcttaggggagaaagttggtttagctttgttaatagagctaatttctcagatttagaaaatgcaatacctaatcctagaccgtcttggtttttaaataatatgattatatctactggttcacttacattgccggttagcccaagtactgatagagcgagggtatggtatggaagtcgagatcgaatttcccctgctaattcacaatttattactgaactaatctctggacaacatacgactgctacacaaactattttagggcgaaatatatttagagtagattctcaagcttgtaatttaaatgataccacatatggagtgaatagggcggtattttatcatgatgcgagtgaaggttctcaaagatccgtgtacgaggggtatattcgaacaactgggatagataaccctagagttcaaaatattaacacttatttacctggagaaaattcagatatcccaactccagaagactatactcatatattaagcacaacaataaatttaacaggaggacttagacaagtagcatctaatcgccgttcatctttagtaatgtatggttggacacataaaagtctggctcgtaacaataccattaatccagatagaattacacagataccattgacgaaggttgatacccgaggcacaggtgtttcttatgtgaatgatccaggatttataggaggagctctacttcaaaggactgaccatggttcgcttggagtattgagggtccaatttccacttcacttaagacaacaatatcgcattagagtccgttatgcttctacaacaaatattcgattgagtgtgaatggcagtttcggtactatttctcaaaatctccctagtacaatgagattaggagaggatttaagatacggatcttttgctataagagagtttaatacttctattagacccactgcaagtccggaccaaattcgattgacaatagaaccatcttttattagacaagaggtctatgtagatagaattgagttcattccagttaatccgacgcgagaggcgaaagaggatctagaagcagcaaaaaaagcggtggcgagcttgtttacacgcacaagggacggattacaagtaaatgtgaaagattatcaagtcgatcaagcggcaaatttagtgtcatgcttatcagatgaacaatatgggtatgacaaaaagatgttattggaagcggtacgtgcggcaaaacgacttagccgagaacgcaacttacttcaggatccagattttaatacaattaatagtacagaagaaaatggatggaaagcaagtaacggcgttactattagtgagggcgggccattctataaaggccgtgcaattcagctagcaagcgcacgagaaaattatccaacatacatttatcaaaaagtagatgcatcggagttaaagccatatacacgctatagactggatggattcgtgaagagtagtcaagatttagaaattgatctcattcaccatcataaagtccatcttgtgaaaaatgtaccagataatttagtacttgatacttacccagatgattcctgcaacggaattaaccgttgtgatgaacagaagatggtaaatgcgcaactggaaacagaacatcatcatccgatggattgctgtgaagcggctcaaacacatgagttttcttcctatattaatacaggcgatctaaatgcaagtgtagatcaaggcatttgggttgtattgaaagttcgaacaacagatggttatgcgacgctaggaaatcttgaattggtagaggtcggaccgttatcgggtgaatctctagaacgtgaacaaagggataatgcgaaatggagtgcagagctaggaagaaagcgtgcagaaacagagagagtatattatgctgccaaacaatccatcaatcatttatttgtggattatcgagatcaacaattaaatccacaaatagggatggcagatattatggacgctcaaaatcttgtcgcatcaatttcagatgtatatagcgatgccgtactgcaaatccctggaattaactatgagatttacacagagctatccaatcgcttacaacaagcatcgtatctgcatatgtctcgaaatgcgatgcaaaatggggactttaacagcggtctagatagttggaatgcaacagcgggtgctacggtacaacaggatggcaatacgcatttcttagttctttctcattgggatgcacaagtttctcaacaatttagagtgcagccgaattgtaaatatgtattacgtgtaacagcagagaaagtaggcggcggagacggatacgtgacaatccgggatggtgctcatcatacagaaacgcttacatttaatgcatgtgattatgatataaatggcacgtacgtgactgataatacgtatctaacaaaagaagtggtattccatccggagacacaacatatgtgggtagaggtaagtgaaacagaaggtgttttccatatagacagtgttgagttcatggaaacccaacagtaa

SEQ ID NO: 3 - DNA, 3471 bp, Bacillus thuringiensis
atgaatcaaaataaacacggaattattggcgcttccaattgtggttgtgcatctgatgatgttgcgaaatatcctttagccaacaatccatattcatctgctttaaatttaaattcttgtcaaaatagtagtattctcaactggattaacataataggcgatgcagcaaaagaagcagtatctattgggacaaccatagtctctcttatcacagcaccttctcttactggattaatttcaatagtatatgaccttataggtaaagtactaggaggtagtagtggacaatccatatcagatttgtctatatgtgacttattatctattattgatttacgggtaagtcagagtgtcttaaatgatgggattgcagattttaatggttctgtactcttatacaggaactatttagaggctctggatagctggaataagaatcctaattctgcttctgctgaagaactccgtactcgttttagaatcgccgactcagaatttgatagaattttaacccgagggtctttaacgaatggtggctcgttagctagacaaaatgcccaaatattattattaccttcttttgcgagcgctgcatttttccatttattactactaagggatgctactagatatggcactaattgggggctatacaatgctacaccttttataaattatcaatcaaaactagtagagcttattgaactatatactgattattgcgtacattggtataatcgaggtttcaacgaactaagacaacgaggcactagtgctacagcttggttagaatttcatagatatcgtagagagatgacattgatggtattagatatagtagcatcattttcaagtcttgatattactaattacccaatagaaacagattttcagttgagtagggtcatttatacagatccaattggttttgtacatcgtagtagtcttaggggagaaagttggtttagctttgttaatagagctaatttctcagatttagaaaatgcaatacctaatcctagaccgtcttggtttttaaataatatgattatatctactggttcacttacattgccggttagcccaagtactgatagagcgagggtatggtatggaagtcgagatcgaatttcccctgctaattcacaatttattactgaactaatctctggacaacatacgactgctacacaaactattttagggcgaaatatatttagagtagattctcaagcttgtaatttaaatgataccacatatggagtgaatagggcggtattttatcatgatgcgagtgaaggttctcaaagatccgtgtacgaggggtatattcgaacaactgggatagataaccctagagttcaaaatattaacacttatttacctggagaaaattcagatatcccaactccagaagactatactcatatattaagcacaacaataaatttaacaggaggacttagacaagtagcatctaatcgccgttcatctttagtaatgtatggttggacacataaaagtctggctcgtaacaataccattaatccagatagaattacacagataccattgacgaaggttgatacccgaggcacaggtgtttcttatgtgaatgatccaggatttataggaggagctctacttcaaaggactgaccatggttcgcttggagtattgagggtccaatttccacttcacttaagacaacaatatcgcattagagtccgttatgcttctacaacaaatattcgattgagtgtgaatggcagtttcggtactatttctcaaaatctccctagtacaatgagattaggagaggatttaagatacggatcttttgctataagagagtttaatacttctattagacccactgcaagtccggaccaaattcgattgacaatagaaccatcttttattagacaagaggtctatgtagatagaattgagttcattccagttaatccgacgcgagaggcgaaagaggatctagaagcagcaaaaaaagcggtggcgagcttgtttacacgcacaagggacggattacaagtaaatgtgaaagattatcaagtcgatcaagcggcaaatttagtgtcatgcttatcagatgaacaatatgggtatgacaaaaagatgttattggaagcggtacgtgcggcaaaacgacttagccgagaacgcaacttacttcaggatccagattttaatacaattaatagtacagaagaaaatggatggaaagcaagtaacggcgttactattagtgagggcgggccattctataaaggccgtgcaattcagctagcaagcgcacgagaaaattatccaacatacatttatcaaaaagtagatgcatcggagttaaagccatatacacgctatagactggatggattcgtgaagagtagtcaagatttagaaattgatctcattcaccatcataaagtccatcttgtgaaaaatgtaccagataatttagtacttgatacttacccagatgattcctgcaacggaattaaccgttgtgatgaacagaagatggtaaatgcgcaactggaaacaggacatcatcatccgatggattgctgtgaagcggctcaaacacatgagttttcttcctatattaatacaggcgatctaaatgcaagtgtagatcaaggcatttgggttgtattgaaagttcgaacaacagatggttatgcgacgctaggaaatcttgaattggtagaggtcggaccgttatcgggtgaatctctagaacgtgaacaaagggataatgcgaaatggagtgcagagctaggaagaaagcgtgcagaaacagagagagtatattatgctgccaaacaatccatcaatcatttatttgtggattatcaagatcaacaattaaatccacaaatagggatggcagatattatggacgctcaaaatcttgtcgcatcaatttcagatgtatatagcgatgccgtactgcaaatccctggaattaactatgagatttacacagagctatccaatcgcttacaacaagcatcgtatctgcatacgtctcgaaatgcgatgcaaaatggggactttaacagcggtctagatagttggaatgcaacagcgggtgctacggtacaacaggatggcaatacgcatttcttagttctttctcattgggatgcacaagtttctcaacaatttagagtgcagccgaattgtaaatatgtattacgtgtaacagcagagaaagtaggcggcggagacggatacgtgacaatccgggatggtgctcatcatacagaaacgcttacatttaatgcatgtgattatgatataaatggcacgtacgtgactgataatacgtatctaacaaaagaagtggtattccatccggagacacaacatatgtgggtagaggtaagtgaaacagaaggtgttttccatatagacagtgttgagttcatggaaacccaacagtaa

SEQ ID NO: 4 - DNA, 3459 bp, Bacillus thuringiensis
atgaatcgaaataatccaaatgaatatgaaattattgatgccccctattgtgggtgtccgtcagatgatgatgtgaggtatcctttggcaagtgacccaaatgcagcgttccaaaatatgaactataaagagtatttacaaacgtatgatggagactacacaggttctcttatcaatcctaacttatctattaatcctagagatgtactacaaacaggtattaatattgtgggaagaatactagggtttttaggtgttccatttgcgggtcaactagttactttctatacctttctcttaaatcagttgtggccaactaatgataatgcagtatgggaagcttttatggcgcaaatagaagagctaatcgatcaaaaaatatcggcgcaagtagtaaggaatgcactcgatgacttaactggattacacgattattatgaggagtatttagcagcattagaggagtggctggaaagaccgaacggagcaagagctaacttagttacacagaggtttgaaaacctgcatactgcatttgtaactagaatgccaagctttggtacgggtcctggtagtcaaagagatgcggtagcgttgttgacggtatatgcacaagcagcgaatttgcatttgttattattaaaagatgcagaaatctatggggcaagatggggacttcaacaagggcaaattaacttatattttaatgctcaacaagaacgtactcgaatttataccaatcattgcgtggaaacatataatagaggattagaagatgtaagaggaacaaatacagaaagttggttaaattaccatcgattccgtagagagatgacattaatggcaatggatttagtggccttattcccatactataatgtgcgacaatatccaaatggggcaaatccacagcttacacgtgaaatatatacggacccaatcgtatataatccaccagctaatcagggaatttgccgacgttgggggaataatccgtataatacattttctgaacttgaaaatgcttttattcgcccgccacatctttttgataggttgaatagattaactatttctagaaaccgatatacagctccaacaactaatagctacctagactattggtcaggtcatactttacaaagccagtatgcaaataacccgacgacatatgaaactagttacggtcagattacctctaacacacgtttattcaatacgactaatggagccaatgcaatagattcaagggcaagaaattttggtaacttatacgctaatttgtatggcgttagcagcttgaacattttcccaacaggtgtgatgagtgaaatcacctcagcccctaatacgtgttggcaagaccttactacaactgaggaactaccactagtgaataataattttaatcttttatctcatgttactttcttacgcttcaatactactcagggtggcccccttgcaactgtagggtttgtacccacatatgtgtggacacgtcaagatgtagattttaataatataattactcccaatagaattactcaaataccagtggtaaaggcatatgagctaagtagtggtgctactgtcgtgaaaggtccaggattcacaggaggagatgtaatccgaagaacaaatactggtggattcggagcaataagggtgtcggtcactggaccgctaacacaacgatatcgcataaggttccgttatgcttcgacaatagattttgatttctttgtaacacgtggaggaactactataaataattttagatttacacgtacaatgaacaggggacaggaatcaagatatgaatcctatcgtactgtagagtttacaactccttttaactttacacaaagtcaagatataattcgaacatctatccagggacttagtggaaatggggaagtataccttgatagaattgaaatcatccctgtaaatccaacacgagaagcggaagaggatttagaagcggcgaagaaagcggtggcgagcttgtttacacgcacaagggacggattacaagtaaatgtgacagattatcaagtcgatcaagcggcaaatttagtgtcatgcttatcagatgaacaatatgcgcatgataaaaagatgttattggaagcggtacgcgcggcaaaacgcctcagccgagaacgtaacttacttcaggacccagattttaatacaatcaatagtacagaagaaaatggatggaaagcaagtaacggcgttactattagtgagggcggtccattctataaaggccgtgcacttcagctagcaagtgcacgagaaaattacccaacatacatctatcaaaaagtagatgcatcggagttaaaaccttatacacgatatagactggatgggttcgtgaagagtagtcaagatttagaaattgatctcattcaccatcataaagtccatcttgtgaaaaatgtactagataatttagtatctgatacttacccagatgattcttgtagtggaatcaatcgatgtgaggaacaacagatggtaaatgcgcaactggaaacagaacatcatcatccgatggattgctgtgaagcagctcaaacacatgagttttcttcctatattgatacaggggatttaaattcgactgtagaccagggaatctgggtgatctttaaagttcgaacaacagatggttatgcgacgctaggaaatcttgaattggtagaggtcggaccgttattgggtgaacctctagaacgtgaacaaagagaaaatgcgaaatggaatgcagagttaggaagaaaacgtgcagaaacagatcgcgtgtatcaagatgccaaacaatccatcaatcatttatttgtggattatcaagatcaacaattaaatccacaaatagggatggcagatattatggacgctcaaaatcttgtcgcatcaatttcagatgtatatagcgatgcagtactgcaaatccctggaattaactatgagatttacacagagctgtccaatcgcttacaacaagcatcgtatctgtatacgtctcgaaatgcggtgcaaaatggggactttaacaacgggctagatagctggaatgcaacagcgggtgcatcggtacaacaggatggcaatacgcatttcttagttctttctcattgggatgcacaagtttcccaacaatttagagtgcagccgaattgtaaatatgtattacgtgtaacagcagagaaagtaggcggcggagacggatacgtgactatccgggatggtgctcatcatacagaaacgcttacatttaatgcatgtgattatgatataaatggcacgtacgtgactgataatacgtatctaacaaaagaagtgatattctattcacatacagaacacatgtgggtagaggtaaatgaaacagaaggtgcatttcatatagatagtattgaattcgttgaaacagaaaagtaa

SEQ ID NO: 5 - DNA, 3468 bp, Bacillus thuringiensis
atgaatcgaaataatcaagatgaatatgaaattattgacgcttccacttgtggttgttcgtcagatgatgttgttcaataccctttggcaagagatccgaatgctgtattccaaaatatgcattataaagattatttgcaaacgtatgatggagactatacaggttctcttataaatcctaacttatctattaatcctagagatgtactgcaaactggaattaatattgtgggaagattactaggatttctaggtgttccatttgctggtcagttagttactttctatacctttcttttaaatcaactgtggccaacaaatgataatgcagtatgggaagcttttatggcacaaatagaagagcttattaatcaaagaatatccgaagcagtagtagggacagcagcggatcatttaacgggattacacgataattatgagttatatgtagaggcattggaggaatggctggaaagaccgaatgctgctagaactaatctactttttaatagatttaccaccctagatagtctttttacacaatttatgccaagctttggtactggacctggaagtcaaaactacgcagttccattacttacagtatacgcacaagcagcgaaccttcatttgttattattaaaggatgctgaaatatatggagcaagatggggactgaaccaaaatcagattaactcattccatacgcgccaacaagaacgtactcaatattatacaaatcattgcgtaacgacgtataataccggtttagatagattaagaggcacaaatactgaaagttggttaaattatcatcgtttccgtagagagatgacattaatggcaatggatttagtagcgctattcccatattataatgtacgacaatatccaaatggagcaaatcctcagcttacacgtgaaatatatacagatccaattgtatttaatccaccagctaatgtgggattatgtagacgttggggcaataacccatataatagattttctgaactagaaaacgcttttatccgcccgccacatctttttgatagattgaataccttaacaattagtagaaatagatttgacgttgggtcaaactttatagaaccgtggtctggacatacgttacgccgtagttattcgaataattcgacagtatatgaagatagttatggccaaattacagccacaagaacaacaattaatctgccggctaatggaactggccgagtagaatcaacagcagtagattttcgtagcgcgcttgtggggatatacggtgttaatagagcttcttttattccaggtggtgtgtttagtggcacgactcagccttctactggaggatgtagagatttgtatgattcaagtgatgaattaccaccagacgaaagtactggaagttttgcccatagactatctcatgttacctttttaagttttacaactaatcaggccggttccatagccaattcaggacgcgtccctacttatgtctggacccatcgcgatgtggactttaataatacaattaaccccaatagaattactcaaataccagtggtaaaggcatatgagctaagtagtggtgctactgtcgtgaaaggtccaggattcacaggaggagatgtaatccgaagaacaaatattggtgggttcggagcaataagggtgtcggtcactggaccgctaacacaacgatatcgcataaggttccgttatgcttcgacaatagattttgatttctttgtaacacgtggaggaactactataaataattttagatttacacgtacaatgaacaggggacaggaatcaagatatgaatcctatcgtactgtagagtttacaactccttttaactttacacaaagtcaagatataattcgaacatctatccagggacttagtggaaatggggaagtataccttgatagaattgaaatcatccctgtaaatccaacacgagaagcggaagaggatctagaagcagcgaagaaagcggtggcgagcttgtttacacgtacaagggacggattacaagtaaatgtgacagattatcaagtcgatcaagcggcaaatttagtgtcatgcttatcagatgaacaatatgggcatgacaaaaagatgttattggaagcggtaagagcggcaaaacgcctcagccgagaacgcaacttacttcaagatccagattttaatacaatcaatagtacagaagaaaatggatggaaagcaagtaacggcgttactattagcgagggcggtccattctataaaggccgtgcgcttcagctagcaagcgcaagagaaaattacccaacatacatttatcaaaaagtaaatgcatcagagttaaagccgtatacacgttatagactggatgggttcgtgaagagtagtcaagatttagaaattgatctcattcaccatcataaagtccatctcgtgaaaaatgtaccagataatttagtatccgatacttactcggatggttcttgcagtggaatgaatcgatgtgaggaacaacagatggtaaatgcgcaactggaaacagaacatcatcatccgatggattgctgtgaagcggctcaaacacatgagttttcttcctatattaatacaggcgatctaaattcaagtgtagatcaaggcatttgggttgtattgaaagttcgaacaaccgatggttatgcgacgctaggaaatcttgaattggtagaggtcggaccgttatcgggtgaatctctagaacgtgaacaaagggataatgcgaaatggagtgcagagctaggaagaaagcgtgcagaaacagatcgcgtgtatcaagatgccaaacaatccatcaatcatttatttgtggattatcaagatcaacaattaaatccagaaatagggatggcagatattattgacgctcaaaatcttgtcgcatcaatttcagatgtgtatagcgatgcagtactgcaaatccctggaattaactatgagatttacacagagctatccaatcgcttacaacaagcatcgtatctgtatacgtctcgaaatgcggtgcaaaatggggactttaacagcggtctagatagttggaatgcaacagggggggctacggtacaacaggatggcaatacgcatttcttagttctttctcattgggatgcacaagtttctcaacaatttagagtgcagccgaattgtaaatatgtattacgtgtaacagcagagaaagtaggcggcggagacggatacgtgacaatccgggatggtgctcatcatacagaaaagcttacatttaatgcatgtgattatgatataaatggcacgtacgtgactgataatacgtatctaacaaaagaagtggtattctattcacatacagaacacatgtgggtagaggtaagtgaaacagaaggtgcatttcatatagatagtattgaattcgttgaaacagaaaagtaa

SEQ ID NO: 6 - DNA, 3471 bp, Artificial Sequence
  Synthetic Cry Gene
atgaatcagaacaagcacggcatcattggggcctcgaactgcggctgcgcctccgacgatgtggctaagtaccctctcgctaacaacccttactccagcgccctgaacctcaattcctgccagaactcgtctatcctcaattggattaacatcattggggacgccgcgaaggaggctgtcagcatcggcaccacgattgtttcactgatcacggccccgtccctgacaggcctcatcagcattgtgtacgacctcatcgggaaggtcctaggcgggtcatccggccagagcatttcggacctgtcgatctgcgatctcctgtctatcattgacctcagggtgtctcagtcagtcctgaacgacgggatcgccgatttcaatggctcagtgctcctgtaccgcaactacctggaggcgctcgactcctggaacaagaatcccaactccgctagcgctgaggagctgaggaccaggttcaggattgccgactccgagttcgatcgcatcctcactcgcggctcactgaccaatggcggctccctcgcccgccagaacgctcagatcctcctgctccctagcttcgcgtcggctgccttcttccacctgctcctgctcagggacgctacgcgctacggaaccaactggggcctctacaatgctactccgttcataaactaccagtccaagctggtcgagctgatcgagctgtacaccgactactgcgttcactggtacaatagggggttcaacgagctgaggcagaggggcacgagcgctacagcttggctggagttccatcgctaccgcagggagatgacgctcatggttctggacatcgtggccagcttcagctcgctcgatattactaactaccctatcgagaccgacttccagctgtcgcgcgtgatttacaccgacccgatcgggttcgtccaccgctcttcactgaggggcgagtcttggttctcattcgtcaatagggcgaacttctcggacctcgagaatgctatcccgaacccccggccatcttggttcctgaacaatatgatcatttccactggcagcctgaccctccccgtttcgccatctacggatcgcgcgagggtgtggtacggctcacgggaccgcatctcaccggctaactcccagttcattacagagctgatctctggccagcacacaactgctacacagactattctgggccggaatatcttccgcgtggacagccaggcctgcaatctcaacgataccacgtacggcgtcaacagggctgttttctaccatgacgcctcggagggctctcagcgctcagtctacgagggatacatcaggacaactggcatcgataatcctcgggtgcagaatattaacacgtacctcccgggcgagaacagcgacatccctacgccggaggattacacacacattctgtcgaccacaatcaacctcaccggcgggctgaggcaggtcgcttctaacaggcgctccagcctcgttatgtacggctggactcataagtcactggcgcgcaacaacacaatcaaccctgataggatcactcagattccgctcaccaaggtggacactagggggaccggcgtgtcgtacgtcaacgatcccggcttcatcggcggggccctgctccagcgcaccgaccacggctccctcggggttctgcgggtgcagttcccactgcatctccgccagcagtacaggattcgggtccgctacgcgtccacaactaacatccgcctcagcgtgaatgggtcgttcggcacgatctcccagaacctgcccagcacaatgaggctcggggaggacctgcgctacggctccttcgccattcgggagttcaacacgagcatccgccccacagcgtcgccagatcagattaggctcactatcgagccaagcttcatcaggcaggaggtctacgttgaccggatcgagttcattcctgtcaacccgacgagggaggctaaggaggatctggaggctgctaagaaggctgtggctagcctcttcaccaggacgagggacggcctgcaagtgaatgtcaaggactaccaggttgatcaggccgcgaacctcgtgtcctgcctgagcgacgagcagtacggctacgataagaagatgctgctcgaggcggtcagggctgctaagaggctctccagggagaggaacctgctccaggaccctgatttcaatacgatcaacagcacagaggagaacgggtggaaggcgtctaatggcgtgaccatttcagagggcggcccattctacaagggcagggctatccagctggcttcggctcgggagaactaccccacgtacatctaccagaaggtcgacgcctctgagctgaagccatacacacgctaccgcctggatggcttcgtgaagtcgtctcaggacctcgagatcgatctgattcaccatcacaaggtccacctggttaagaatgtgcccgacaacctggtcctcgacacctacccagacgattcctgcaatggcatcaacaggtgcgacgagcagaagatggtgaacgcccagctcgagaccgagcatcaccatccgatggactgctgcgaggcggctcagacgcacgagttctcatcctacattaacacaggggacctgaatgccagcgtggatcagggcatctgggtggtcctcaaagtcaggaccacggacgggtacgctacgctgggcaacctggagctggttgaagtggggccactctcgggcgagtctctggagagggagcagagggacaacgccaagtggagcgctgagctgggcaggaagagggctgagaccgagagggtctactacgccgcgaagcagtcgatcaatcacctcttcgtggactacagggatcagcagctgaacccccagattggcatggctgacatcatggatgcccagaacctcgtcgcgtcaatctccgacgtgtactccgatgcggtcctgcagatcccaggcatcaactacgagatctacacggagctgagcaaccggctgcagcaggcctcgtacctccacatgtctcgcaatgcgatgcagaacggggacttcaattctggcctggattcatggaatgcgactgctggggccaccgttcagcaggacggcaacacccacttcctggtgctctcccattgggatgcccaagttagccagcagttccgcgtgcagccgaactgcaagtacgtcctgagggttactgctgagaaggtcggcgggggcgacggctacgttaccatccgcgatggcgctcaccatacagagactctcaccttcaacgcctgcgactacgatatcaatggcacgtacgtgacagacaacacttacctgaccaaggaggttgtgttccacccggagacccagcatatgtgggtcgaggttagcgagacggagggcgtgttccacatagacagcgttgagttcatggagacccagcagtag

SEQ ID NO: 7 - DNA, 3471 bp, Artificial Sequence; identical to SEQ ID NO: 6
  Synthetic Cry Gene

SEQ ID NO: 8 - DNA, 3471 bp, Artificial Sequence
  Synthetic Cry gene
atgaatcagaacaagcacggcatcattggggcctcgaactgcggctgcgcctccgacgatgtggctaagtaccctctcgctaacaacccttactccagcgccctgaacctcaattcctgccagaactcgtctatcctcaattggattaacatcattggggacgccgcgaaggaggctgtcagcatcggcaccacgattgtttcactgatcacggccccgtccctgacaggcctcatcagcattgtgtacgacctcatcgggaaggtcctaggcgggtcatccggccagagcatttcggacctgtcgatctgcgatctcctgtctatcattgacctcagggtgtctcagtcagtcctgaacgacgggatcgccgatttcaatggctcagtgctcctgtaccgcaactacctggaggcgctcgactcctggaacaagaatcccaactccgctagcgctgaggagctgaggaccaggttcaggattgccgactccgagttcgatcgcatcctcactcgcggctcactgaccaatggcggctccctcgcccgccagaacgctcagatcctcctgctccctagcttcgcgtcggctgccttcttccacctgctcctgctcagggacgctacgcgctacggaaccaactggggcctctacaatgctactccgttcataaactaccagtccaagctggtcgagctgatcgagctgtacaccgactactgcgttcactggtacaatagggggttcaacgagctgaggcagaggggcacgagcgctacagcttggctggagttccatcgctaccgcagggagatgacgctcatggttctggacatcgtggccagcttcagctcgctcgatattactaactaccctatcgagaccgacttccagctgtcgcgcgtgatttacaccgacccgatcgggttcgtccaccgctcttcactgaggggcgagtcttggttctcattcgtcaatagggcgaacttctcggacctcgagaatgctatcccgaacccccggccatcttggttcctgaacaatatgatcatttccactggcagcctgaccctccccgtttcgccatctacggatcgcgcgagggtgtggtacggctcacgggaccgcatctcaccggctaactcccagttcattacagagctgatctctggccagcacacaactgctacacagactattctgggccggaatatcttccgcgtggacagccaggcctgcaatctcaacgataccacgtacggcgtcaacagggctgttttctaccatgacgcctcggagggctctcagcgctcagtctacgagggatacatcaggacaactggcatcgataatcctcgggtgcagaatattaacacgtacctcccgggcgagaacagcgacatccctacgccggaggattacacacacattctgtcgaccacaatcaacctcaccggcgggctgaggcaggtcgcttctaacaggcgctccagcctcgttatgtacggctggactcataagtcactggcgcgcaacaacacaatcaaccctgataggatcactcagattccgctcaccaaggtggacactagggggaccggcgtgtcgtacgtcaacgatcccggcttcatcggcggggccctgctccagcgcaccgaccacggctccctcggggttctgcgggtgcagttcccactgcatctccgccagcagtacaggattcgggtccgctacgcgtccacaactaacatccgcctcagcgtgaatgggtcgttcggcacgatctcccagaacctgcccagcacaatgaggctcggggaggacctgcgctacggctccttcgccattcgggagttcaacacgagcatccgccccacagcgtcgccagatcagattaggctcactatcgagccaagcttcatcaggcaggaggtctacgttgaccggatcgagttcattcctgtcaacccgacgagggaggctaaggaggatctggaggctgctaagaaggctgtggctagcctcttcaccaggacgagggacggcctgcaagtgaatgtcaaggactaccaggttgatcaggccgcgaacctcgtgtcctgcctgagcgacgagcagtacggctacgataagaagatgctgctcgaggcggtcagggctgctaagaggctctccagggagaggaacctgctccaggaccctgatttcaatacgatcaacagcacagaggagaacgggtggaaggcgtctaatggcgtgaccatttcagagggcggcccattctacaagggcagggctatccagctggcttcggctcgggagaactaccccacgtacatctaccagaaggtcgacgcctctgagctgaagccatacacacgctaccgcctggatggcttcgtgaagtcgtctcaggacctcgagatcgatctgattcaccatcacaaggtccacctggttaagaatgtgcccgacaacctggtcctcgacacctacccagacgattcctgcaatggcatcaacaggtgcgacgagcagaagatggtgaacgcccagctcgagaccggacatcaccatccgatggactgctgcgaggcggctcagacgcacgagttctcatcctacattaacacaggggacctgaatgccagcgtggatcagggcatctgggtggtcctcaaagtcaggaccacggacgggtacgctacgctgggcaacctggagctggttgaagtggggccactctcgggcgagtctctggagagggagcagagggacaacgccaagtggagcgctgagctgggcaggaagagggctgagaccgagagggtctactacgccgcgaagcagtcgatcaatcacctcttcgtggactaccaagatcagcagctgaacccccagattggcatggctgacatcatggatgcccagaacctcgtcgcgtcaatctccgacgtgtactccgatgcggtcctgcagatcccaggcatcaactacgagatctacacggagctgagcaaccggctgcagcaggcctcgtacctccacacgtctcgcaatgcgatgcagaacggggacttcaattctggcctggattcatggaatgcgactgctggggccaccgttcagcaggacggcaacacccacttcctggtgctctcccattgggatgcccaagttagccagcagttccgcgtgcagccgaactgcaagtacgtcctgagggttactgctgagaaggtcggcgggggcgacggctacgttaccatccgcgatggcgctcaccatacagagactctcaccttcaacgcctgcgactacgatatcaatggcacgtacgtgacagacaacacttacctgaccaaggaggttgtgttccacccggagacccagcatatgtgggtcgaggttagcgagacggagggcgtgttccacatagacagcgttgagttcatggagacccagcagtag

SEQ ID NO: 9 - DNA, 3459 bp, Artificial Sequence
  Synthetic Cry Gene
atgaacaggaacaacccaaacgagtacgagattattgatgctccatactgcggctgcccctccgatgacgatgtgcgctaccccctcgccagcgacccgaacgccgcgttccagaatatgaactacaaggagtacctgcagacctacgacggcgattacacggggtcactgattaatccaaacctctccatcaatcctcgcgacgtcctccagaccggaatcaacattgttggccgcatcctcggcttcctgggcgtgccgttcgctggccagctggttaccttctacacgttcctcctgaaccagctctggcctacgaatgacaacgcggtgtgggaggccttcatggcgcagatcgaggagctgattgatcagaagatctccgctcaggtggtcaggaacgccctcgacgatctgaccggcctccacgactactacgaggagtacctggctgctctcgaggagtggctcgagaggccaaacggcgctcgcgctaatctggtcacgcagcgcttcgagaacctccataccgccttcgtgacgaggatgccgagcttcgggacaggccccgggtcgcagagggacgcggttgctctcctgactgtgtacgcgcaggcggctaacctgcacctcctgctcctgaaggatgctgagatctacggcgctcggtgggggctgcagcagggccagatcaacctctacttcaatgcccagcaggagcgcacaaggatctacactaaccactgcgttgagacctacaatagggggctcgaggacgtgcggggcacgaacacagagagctggctgaattaccatcgcttccgcagggagatgacgctcatggcgatggacctcgtggcgctcttcccctactacaacgtccgccagtacccaaatggcgccaaccctcagctgacaagggagatctacactgacccgatcgtgtacaacccaccagctaatcaggggatctgcaggcgctggggcaacaatccctacaacaccttctctgagctggagaatgcgttcattaggccacctcacctcttcgaccgcctgaacaggctcaccatctcccggaatcgctacacggctccaaccacgaactcgtacctggattactggtctggccataccctccagtcacagtacgcgaacaatcctacaacttacgagacgtcctacggccagattacaagcaacactcgcctcttcaataccacgaacggcgctaatgctatcgacagcagggcccggaacttcgggaatctgtacgcgaatctctacggcgtctccagcctgaacattttcccaaccggcgttatgtcagagatcacctccgcccctaacacgtgctggcaggacctcacaactaccgaggagctgccactggtgaacaataacttcaatctcctgtcccacgtcacattcctgaggttcaacacgacacagggcggcccactcgcgactgttggcttcgtgcccacctacgtgtggacgcggcaggacgtcgatttcaataacatcattacaccaaaccgcatcactcagattcctgttgtgaaggcgtacgagctgtcgtctggcgctacagtcgttaagggcccggggttcactggcggggacgtcattaggaggactaacaccggcgggttcggggctatcagggtgagcgtcacaggccccctcactcagcgctacaggattcggttccgctacgcgtcgaccatcgacttcgatttcttcgtcacgcgcggcgggactaccatcaataacttccggttcacgcgcaccatgaacaggggccaggagagccggtacgagtcgtaccgcaccgtggagttcacgacaccgttcaacttcacacagagccaggacatcattcgcacttctattcagggcctgtcaggcaacggggaggtttacctcgaccggatcgagatcattccagtgaacccaaccagggaggctgaggaggatctcgaggctgcgaagaaggctgtggcctcgctgttcactaggacccgggacggcctccaggttaatgtgacggactaccaggtggatcaggctgccaacctggtctcgtgcctctctgacgagcagtacgctcacgataagaagatgctcctggaggccgtccgcgctgctaagaggctgtcgagggagaggaacctcctgcaggacccagatttcaacaccattaattctacggaggagaacgggtggaaggcgtcgaatggcgtgaccatctctgagggcgggcctttctacaagggccgcgctctccagctggcttcagctagggagaactacccgacatacatctaccagaaggtcgacgcctccgagctgaagccctacacgcgctaccgcctcgatggcttcgtgaagtcatcccaggacctggagatcgatctcattcaccatcacaaggtccacctggttaagaacgtgctggacaatctcgtcagcgatacctacccggacgattcttgctcaggcatcaatcgctgcgaggagcagcagatggtgaacgcccagctcgagaccgagcatcaccatccgatggactgctgcgaggctgctcagacgcatgagttcagctcgtacatcgacacaggggatctgaactccactgtggaccagggcatctgggtcatcttcaaggtgcgcactaccgatgggtacgcgaccctcggcaacctcgagctggtcgaggttgggccgctcctgggcgagccactggagagggagcagagggagaacgctaagtggaatgctgagctgggcaggaagcgggctgagaccgaccgcgtctaccaggatgctaagcagtccatcaatcacctgttcgtggactaccaggatcagcagctcaacccacagattggcatggctgacatcatggatgcccagaacctggtcgcgtccatcagcgacgtctactctgatgccgttctccagatccctggcattaattacgagatctacacagagctgtcaaaccggctccagcaggcctcctacctgtacactagccgcaacgcggtgcagaatggggacttcaataacggcctcgattcctggaatgctacagctggggctagcgtccagcaggacggcaacactcacttcctcgttctgtctcattgggatgcccaggtttcacagcagttcagggtgcagccgaactgcaagtatgtgctgagggttaccgctgagaaggttggcgggggcgacggctacgtgacgatcagggatggcgctcaccatacggagacactgactttcaacgcctgcgactacgatatcaatggcacctacgtcacggacaacacatacctcactaaggaggtcatattctacagccacaccgagcatatgtgggtggaggtcaacgagacggagggcgccttccacatagactcgattgagttcgtggagaccgagaagtga

SEQ ID NO: 10 - DNA, 3468 bp, Artificial Sequence
  Synthetic Cry Gene
atgaataggaataaccaggacgagtacgagatcattgacgcttcgacttgcgggtgcagctcagacgatgttgttcagtaccccctcgctcgcgatcccaatgccgtgttccagaacatgcactacaaggactacctccagacatacgacggcgattacactgggtcgctcattaacccaaatctgtctatcaatcctcgcgacgtcctgcagacgggaatcaacattgttgggaggctcctgggcttcctcggggttccgttcgctggccagctggtgacattctacactttcctcctgaaccagctctggcccaccaacgacaatgcggtctgggaggccttcatggcgcagatcgaggagctgattaaccagcgcatctccgaggctgtggtcggcaccgctgctgatcacctcacggggctgcatgacaactacgagctttacgtggaggctctcgaggagtggctggagaggccaaacgctgctaggacgaacctcctgttcaataggttcaccacgctcgactccctgttcacacagttcatgccatcattcgggactggccccggctcccagaactacgccgtccctctcctgaccgtttacgcgcaggcggctaacctccacctcctgctcctgaaggacgctgagatctacggcgctcgctgggggctgaaccagaatcagatcaacagcttccacacaaggcagcaggagcggacccagtactacacgaatcattgcgtgacaacttacaacaccggcctcgataggctgagggggaccaatacggagtcctggctcaactaccataggttccgcagggagatgaccctgatggcgatggacctcgtggcgctgttcccgtactacaacgtccggcagtacccaaacggcgctaatccacagctcacccgcgagatctacacggacccaatcgtcttcaacccaccagctaatgttggcctgtgcaggcgctgggggaacaatccttacaatcgcttcagcgagctggagaacgccttcatcaggccacctcacctgttcgatcggctcaatacactgactatttcgaggaaccggttcgacgtcggcagcaatttcatcgagccgtggtcgggccatacgctgaggaggtcctacagcaacaattcaacagtgtacgaggattcctacggccagattaccgctacgaggaccacgatcaacctccctgccaatggcacagggcgggtggagtctactgctgtcgacttccgctcagccctggttggcatctacggggtgaacagggcgagcttcatcccgggcggggtcttcagcggcacaactcagccatcgaccggcgggtgcagggacctctacgattccagcgacgagctgccaccagacgagagcacgggctcgttcgctcacaggctctctcatgtcacattcctgtcattcaccacgaaccaggctggctcgatcgccaattctgggagggttccgacatacgtgtggactcaccgggacgtggatttcaacaataccatcaacccaaatcgcatcacgcagattcctgttgtgaaggcgtacgagctgtcctccggcgctaccgtcgttaagggcccggggttcacgggcggggacgtgattcgcaggacaaacatcggcgggttcggcgctatcagggtctccgttaccggccccctgacgcagcgctacaggattcggttccgctacgcctccactatcgacttcgatttcttcgtcacccggggcgggacaactatcaacaatttccgcttcacaaggactatgaacaggggccaggagtcacggtacgagtcctaccgcaccgtggagttcaccacgcccttcaacttcacgcagtcccaggacatcattaggacatccattcagggcctcagcggcaacggggaggtttacctggatcgcatcgagatcattccagtgaaccctacgagggaggctgaggaggacctcgaggctgcgaagaaggctgtggctagcctcttcaccaggacgagggatggcctgcaagtgaatgtcaccgattaccaggtggaccaggctgccaacctcgtctcttgcctgtcagatgagcagtacggccacgacaagaagatgctcctggaggccgtccgcgctgctaagaggctgtccagggagaggaacctcctgcaggacccagatttcaacacaatcaatagcactgaggagaatggctggaaggcgtccaacggggtgaccatcagcgagggcgggcctttctacaagggccgcgctctccagctggcttcggctagggagaattacccaacttacatctaccagaaggtcaacgcctctgagctgaagccttacacgcgctaccgcctggatggcttcgtgaagtcatcccaggatctcgagatcgacctgattcaccatcacaaggtgcacctcgtcaagaacgttccggacaatctggtcagcgatacgtactcggacggctcgtgctctgggatgaatcgctgcgaggagcagcagatggtgaacgcgcagctcgagacagagcatcaccatccgatggactgctgcgaggccgcgcagactcatgagttcagctcgtacattaataccggcgatctgaactcttcagtcgaccagggcatctgggtggtcctcaaggttcgcacaactgatggctacgccacgctggggaacctcgagctggttgaagtgggcccactctccggggagagcctggagagggagcagagggacaacgcgaagtggtccgctgagctgggcaggaagcgggctgagaccgatagggtttaccaggacgctaagcagtccatcaatcacctcttcgtggattaccaggaccagcagctgaacccggagattggcatggctgatatcattgacgcccagaacctcgtcgcgtcaatctccgatgtctacagcgacgccgttctgcagatccccggcattaattacgagatctacacggagctgtcgaacaggctgcagcaggcctcgtacctctacacatctcggaacgcggtgcagaatggcgatttcaactctgggctggactcatggaatgctaccggcggggctacggtgcagcaggatggcaacacccacttcctcgtcctgtcccattgggacgctcaggtgagccagcagttccgggtccagccgaactgcaagtatgtgctgagggtcactgctgagaaggttggcgggggcgatggctacgtgaccatcagggacggggctcaccatacagagaagctcactttcaacgcctgcgactacgatatcaatggcacctacgtcacggacaacacatacctaactaaggaggttgtgttctactcgcacactgagcatatgtgggtcgaggtttctgagaccgagggcgccttccacatagactcaattgagttcgtggagaccgagaagtga

SEQ ID NO: 11 - DNA, 3507 bp, Artificial Sequence
  Synthetic Cry Gene
atgaataggaataaccagaacgagtacgaggtcattgatgctccccattgcggctgcccggcggacgatgttgtgaagtacccactgaccgacgatccgaacgccggcctgcagaacatgaattacaaggagtacctccagacctacggcggggactacaccgacccgctgatcaaccctaatctctcggtttctggcaaggacgtgattcaggtcggaatcaacattgtggggcgcctcctgtccttcttcgggttcccattctccagccagtgggtgacagtctacacttacctcctgaattcactgtggcctgacgatgagaactccgtttgggacgccttcatggagcgggtggaggagctgatcgatcagaagattagcgaggctgtcaagggccgcgcgctcgacgatctgaccgggctccagtacaactacaacctctacgtggaggcgctggacgagtggctcaacaggccaaatggcgctcgggcctctctcgtgtcacagaggttcaacatcctggattccctcttcacccagttcatgccatccttcgggagcggccccgggagccagaattacgcgacgatcctcctgcctgtgtacgctcaggccgcgaacctgcacctcctgctcctgaaggacgctgatatctacggcgccaggtgggggctcaaccagacccagattgaccagttccactctaggcagcagtcactcacccagacgtacacaaaccattgcgtgacagcctacaatgacggcctggctgagctgagggggacttcggtcgcctcttggctgaagtaccaccagtaccgcagggagatgactgtcaccgcgatggacctggttgctctcttcccatactacaacgtgcgccagtacccgaacggcgcgaatccccagctcaccagggaggtgtacacggacccaatcgtcttcaacccaccagagaggccttctggcgctttctgcgagtcattctacaccatcagggctgctagggagaggctgacgttctcccagctcgagcacgcgatcattcgcccacctaggctgttcgagcggttccaggctctcggcatctacacaggggaggcccgcctcaacgctaattccgccccgatgaattactggatcggccatttcattaggaacacgaggctgggggacagcaccacgatcacaactaattacggcaccacgaacaataggctcaccaacttctcaatgccctccgacgtctaccagatcaactccacgtcgtctaatctcgcggctattctgggcacactctacggggtgactcgcgcccagttccacttcggctcagggtccttcagcacctacgtgggccagaacagcgtcctgccgcagtgccatcagaactacaatagcatcgaggagctgccaaaccagtcggacgagcctaccgttcgctcgtactctcacaggctgtcccatatcacgagcttcaacttcaatgtgcagctgaacaatccgctcatttctgcgggcaacatgcccgtttacgtgtggacccacaggtcagtcgacctgacgaaccggatctcatccgatcgcatcacccagattccggtggtcaaggcttacgagctgtcctccggcgctacagttgtgaagggccccgggttcactggcggggacgtgatcaggaggacgaacacaggcgggttcggcgcgattagggtctcggttaccgggccgctcacgcagcgctaccgcatccgcttccgctacgcttctaccattgacttcgatttcttcgtcacgcggggcgggacaactatcaacaatttcaggttcactcggaccatgaacaggggccaggagtcgcggtacgagtcttaccgcaccgtggagttcaccacgcccttcaacttcacacagtcccaggacatcattcgcacttcaatccagggcctgtccggcaatggggaggtctacctcgaccgcattgagatcattccggttaaccccacgagggaggctgaggaggatctggaggctgcgaagaaggcggtggctagcctgttcacgaggacacgggacggcctccaagtgaatgtcaaggactaccaggtcgatcaggctgccaacctggttagctgcctctcggacgagcagtacggctacgataagaagatgctcctggaggccgtgcgcgctgctaagaggctctcgagggagaggaacctcctgcaggacccggatttcaacacaatcaattctactgaggagaacggctggaaggcttccaatggggtgaccattagcgagggcggcccattctacaagggcagggccctccagctggcttcagctcgggagaactacccaacatacatctaccagaaggtcgacgccagcgagctgaagccttacactcgctaccgcctcgatggcttcgtgaagtcttcacaggacctggagatcgatctcattcaccatcacaaggttcacctggtgaagaacgtcccggacaatctcgtctccgatacgtaccccgacgattcatgctccggcatcaataggtgccaggagcagcagatggtgaacgcccagctggagacagagcatcaccatccgatggactgctgcgaggccgcgcagactcatgagttctccagctacatcgacacaggcgatctgaacagcactgtggaccaggggatctgggtcattttcaaggttaggacaactgatggctacgcgaccctcgggaacctcgagctggttgaagtgggcccactcctgggggagcctctggagagggagcagagggagaacgcgaagtggaatgctgagctgggcaggaagcgggctgagaccgaccgcgtctaccaggatgccaagcagagcatcaatcacctgttcgttgactaccaggatcagcagctcaacccagagatcggcatggccgacattatggatgcgcagaacctggtcgctagcatctcggacgtttactcggatgccgtgctccagatccctggcattaattacgagatctacaccgagctgagcaacaggctccagcaggcgagctacctgtacacgtcgcggaacgctgtgcagaatggcgacttcaacaatgggctcgattcttggaatgctaccgctggcgcttcagtgcagcaggacgggaacacgcacttcctcgtcctgtcgcattgggatgcccaggtttctcagcagttccgggtgcagccgaactgcaagtatgtgctcagggtgacagctgagaaagtgggcgggggcgacggctacgtcactatccgcgacgatgcccaccatactgagaccctgacgttcaacgcgtgcgactacgatatcaatggcacctacgtcacggacaacacatacatcactaaggaggtcgttttctactcccacacagatcatatgtgggtcgaggttagcgagactgagggcgccttccacatcgactcgcttgagttcgtggagaccgagaagtga

SEQ ID NO: 12 - DNA, 3471 bp, Artificial Sequence
  Synthetic Cry Gene
atgaatcagaacaagcacggcatcattggggcctcgaactgcggctgcgcctccgacgatgtggctaagtaccctctcgctaacaacccttactccagcgccctgaacctcaattcctgccagaactcgtctatcctcaattggattaacatcattggggacgccgcgaaggaggctgtcagcatcggcaccacgattgtttcactgatcacggccccgtccctgacaggcctcatcagcattgtgtacgacctcatcgggaaggtcatcggcgggtcatccggccagagcatttcggacctgtcgatctgcgatctcctgtctatcattgacctcagggtgtctcagtcagtcctgaacgacgggatcgccgatttcaatggctcagtgctcctgtaccgcaactacctggaggcgctcgactcctggaacaagaatcccaactccgctagcgctgaggagctgaggaccaggttcaggattgccgactccgagttcgatcgcatcctcactcgcggctcactgaccaatggcggctccctcgcccgccagaacgctcagatcctcctgctccctagcttcgcgtcggctgccttcttccacctgctcctgctcagggacgctacgcgctacggaaccaactggggcctctacaatgctactccgttcataaactaccagtccaagctggtcgagctgatcgagctgtacaccgactactgcgttcactggtacaatagggggttcaacgagctgaggcagaggggcacgagcgctacagcttggctggagttccatcgctaccgcagggagatgacgctcatggttctggacatcgtggccagcttcagctcgctcgatattactaactaccctatcgagaccgacttccagctgtcgcgcgtgatttacaccgacccgatcgggttcgtccaccgctcttcactgaggggcgagtcttggttctcattcgtcaatagggcgaacttctcggacctcgagaatgctatcccgaacccccggccatcttggttcctgaacaatatgatcatttccactggcagcctgaccctccccgtttcgccatctacggatcgcgcgagggtgtggtacggctcacgggaccgcatctcaccggctaactcccagttcattacagagctgatctctggccagcacacaactgctacacagactattctgggccggaatatcttccgcgtggacagccaggcctgcaatctcaacgataccacgtacggcgtcaacagggctgttttctaccatgacgcctcggagggctctcagcgctcagtctacgagggatacatcaggacaactggcatcgataatcctcgggtgcagaatattaacacgtacctcccgggcgagaacagcgacatccctacgccggaggattacacacacattctgtcgaccacaatcaacctcaccggcgggctgaggcaggtcgcttctaacaggcgctccagcctcgttatgtacggctggactcataagtcactggcgcgcaacaacacaatcaaccctgataggatcactcagattccgctcaccaaggtggacactagggggaccggcgtgtcgtacgtcaacgatcccggcttcatcggcggggccctgctccagcgcaccgaccacggctccctcggggttctgcgggtgcagttcccactgcatctccgccagcagtacaggattcgggtccgctacgcgtccacaactaacatccgcctcagcgtgaatgggtcgttcggcacgatctcccagaacctgcccagcacaatgaggctcggggaggacctgcgctacggctccttcgccattcgggagttcaacacgagcatccgccccacagcgtcgccagatcagattaggctcactatcgagccaagcttcatcaggcaggaggtctacgttgaccggatcgagttcattcctgtcaacccgacgagggaggctaaggaggatctggaggctgctaagaaggctgtggctagcctcttcaccaggacgagggacggcctgcaagtgaatgtcaaggactaccaggttgatcaggccgcgaacctcgtgtcctgcctgagcgacgagcagtacggctacgataagaagatgctgctcgaggcggtcagggctgctaagaggctctccagggagaggaacctgctccaggaccctgatttcaatacgatcaacagcacagaggagaacgggtggaaggcgtctaatggcgtgaccatttcagagggcggcccattctacaagggcagggctatccagctggcttcggctcgggagaactaccccacgtacatctaccagaaggtcgacgcctctgagctgaagccatacacacgctaccgcctggatggcttcgtgaagtcgtctcaggacctcgagatcgatctgattcaccatcacaaggtccacctggttaagaatgtgcccgacaacctggtcctcgacacctacccagacgattcctgcaatggcatcaacaggtgcgacgagcagaagatggtgaacgcccagctcgagaccgagcatcaccatccgatggactgctgcgaggcggctcagacgcacgagttctcatcctacattaacacaggggacctgaatgccagcgtggatcagggcatctgggtggtcctcaaagtcaggaccacggacgggtacgctacgctgggcaacctggagctggttgaagtggggccactctcgggcgagtctctggagagggagcagagggacaacgccaagtggagcgctgagctgggcaggaagagggctgagaccgagagggtctactacgccgcgaagcagtcgatcaatcacctcttcgtggactacagggatcagcagctgaacccccagattggcatggctgacatcatggatgcccagaacctcgtcgcgtcaatctccgacgtgtactccgatgcggtcctgcagatcccaggcatcaactacgagatctacacggagctgagcaaccggctgcagcaggcctcgtacctccacatgtctcgcaatgcgatgcagaacggggacttcaattctggcctggattcatggaatgcgactgctggggccaccgttcagcaggacggcaacacccacttcctggtgctctcccattgggatgcccaagttagccagcagttccgcgtgcagccgaactgcaagtacgtcctgagggttactgctgagaaggtcggcgggggcgacggctacgttaccatccgcgatggcgctcaccatacagagactctcaccttcaacgcctgcgactacgatatcaatggcacgtacgtgacagacaacacttacctgaccaaggaggttgtgttccacccggagacccagcatatgtgggtcgaggttagcgagacggagggcgtgttccacctggacagcgttgagttcatggagacccagcagtag

SEQ ID NO: 13 - DNA, 3471 bp, Artificial Sequence
  Synthetic Cry Gene
atgaatcagaacaagcacggcatcattggggcctcgaactgcggctgcgcctccgacgatgtggctaagtaccctctcgctaacaacccttactccagcgccctgaacctcaattcctgccagaactcgtctatcctcaattggattaacatcattggggacgccgcgaaggaggctgtcagcatcggcaccacgattgtttcactgatcacggccccgtccctgacaggcctcatcagcattgtgtacgacctcatcgggaaggtcatcggcgggtcatccggccagagcatttcggacctgtcgatctgcgatctcctgtctatcattgacctcagggtgtctcagtcagtcctgaacgacgggatcgccgatttcaatggctcagtgctcctgtaccgcaactacctggaggcgctcgactcctggaacaagaatcccaactccgctagcgctgaggagctgaggaccaggttcaggattgccgactccgagttcgatcgcatcctcactcgcggctcactgaccaatggcggctccctcgcccgccagaacgctcagatcctcctgctccctagcttcgcgtcggctgccttcttccacctgctcctgctcagggacgctacgcgctacggaaccaactggggcctctacaatgctactccgttcataaactaccagtccaagctggtcgagctgatcgagctgtacaccgactactgcgttcactggtacaatagggggttcaacgagctgaggcagaggggcacgagcgctacagcttggctggagttccatcgctaccgcagggagatgacgctcatggttctggacatcgtggccagcttcagctcgctcgatattactaactaccctatcgagaccgacttccagctgtcgcgcgtgatttacaccgacccgatcgggttcgtccaccgctcttcactgaggggcgagtcttggttctcattcgtcaatagggcgaacttctcggacctcgagaatgctatcccgaacccccggccatcttggttcctgaacaatatgatcatttccactggcagcctgaccctccccgtttcgccatctacggatcgcgcgagggtgtggtacggctcacgggaccgcatctcaccggctaactcccagttcattacagagctgatctctggccagcacacaactgctacacagactattctgggccggaatatcttccgcgtggacagccaggcctgcaatctcaacgataccacgtacggcgtcaacagggctgttttctaccatgacgcctcggagggctctcagcgctcagtctacgagggatacatcaggacaactggcatcgataatcctcgggtgcagaatattaacacgtacctcccgggcgagaacagcgacatccctacgccggaggattacacacacattctgtcgaccacaatcaacctcaccggcgggctgaggcaggtcgcttctaacaggcgctccagcctcgttatgtacggctggactcataagtcactggcgcgcaacaacacaatcaaccctgataggatcactcagattccgctcaccaaggtggacactagggggaccggcgtgtcgtacgtcaacgatcccggcttcatcggcggggccctgctccagcgcaccgaccacggctccctcggggttctgcgggtgcagttcccactgcatctccgccagcagtacaggattcgggtccgctacgcgtccacaactaacatccgcctcagcgtgaatgggtcgttcggcacgatctcccagaacctgcccagcacaatgaggctcggggaggacctgcgctacggctccttcgccattcgggagttcaacacgagcatccgccccacagcgtcgccagatcagattaggctcactatcgagccaagcttcatcaggcaggaggtctacgttgaccggatcgagttcattcctgtcaacccgacgagggaggctaaggaggatctggaggctgctaagaaggctgtggctagcctcttcaccaggacgagggacggcctgcaagtgaatgtcaaggactaccaggttgatcaggccgcgaacctcgtgtcctgcctgagcgacgagcagtacggctacgataagaagatgctgctcgaggcggtcagggctgctaagaggctctccagggagaggaacctgctccaggaccctgatttcaatacgatcaacagcacagaggagaacgggtggaaggcgtctaatggcgtgaccatttcagagggcggcccattctacaagggcagggctatccagctggcttcggctcgggagaactaccccacgtacatctaccagaaggtcgacgcctctgagctgaagccatacacacgctaccgcctggatggcttcgtgaagtcgtctcaggacctcgagatcgatctgattcaccatcacaaggtccacctggttaagaatgtgcccgacaacctggtcctcgacacctacccagacgattcctgcaatggcatcaacaggtgcgacgagcagaagatggtgaacgcccagctcgagaccggacatcaccatccgatggactgctgcgaggcggctcagacgcacgagttctcatcctacattaacacaggggacctgaatgccagcgtggatcagggcatctgggtggtcctcaaagtcaggaccacggacgggtacgctacgctgggcaacctggagctggttgaagtggggccactctcgggcgagtctctggagagggagcagagggacaacgccaagtggagcgctgagctgggcaggaagagggctgagaccgagagggtctactacgccgcgaagcagtcgatcaatcacctcttcgtggactaccaagatcagcagctgaacccccagattggcatggctgacatcatggatgcccagaacctcgtcgcgtcaatctccgacgtgtactccgatgcggtcctgcagatcccaggcatcaactacgagatctacacggagctgagcaaccggctgcagcaggcctcgtacctccacacgtctcgcaatgcgatgcagaacggggacttcaattctggcctggattcatggaatgcgactgctggggccaccgttcagcaggacggcaacacccacttcctggtgctctcccattgggatgcccaagttagccagcagttccgcgtgcagccgaactgcaagtacgtcctgagggttactgctgagaaggtcggcgggggcgacggctacgttaccatccgcgatggcgctcaccatacagagactctcaccttcaacgcctgcgactacgatatcaatggcacgtacgtgacagacaacacttacctgaccaaggaggttgtgttccacccggagacccagcatatgtgggtcgaggttagcgagacggagggcgtgttccacctggacagcgttgagttcatggagacccagcagtag

SEQ ID NO: 14 - DNA, 5919 bp, Artificial Sequence
  Synthetic Cry Gene
atggacctggatgggaataagacagagacagagaccgagattgtgaatgggagcgagagcagcattgacccgagcagcgtttcgtacgctgggaacaatagctactccagcgccctgaacctcaattcgtgccagaataggggcatcgctcagtgggttaacacgctgggcggggctattgggcaggccgtgagcatcggcacatctatcatttcactcctggccgcgccgacactcactgggtctatttcactggccttcaatctcatcaggaggatggggaccggctccaacggctcgtctatttccgacctgagcatctgcgatctcctgagcatcattaacctgcgggtttcgcaggctgtgctcaacgacgggatcgctgatttcaatggctccgttgctgtgtacgacctgtacctccacgccctgcgcagctggaacaataaccctaacgctgctactgctgaggagctgaggacccgcttcaggatcgccgattcggagttcgagaggattctgacgaggggctcgctcacacatggcggctccctcgcccgccaggacgctcaggtcctcctgctcccgtccttcgttaacgcggcttacctgcacctgctcatcctccgcgatgcttcgcgctacggggcctcttggggcctcttcaacaccacgccgcatatcaattaccccgtgaggctgcagcagctcattggcagctacacgcactactgcacacattggtacaaccaggggctgaatgagatccggcagcgcggcaacactgccgtgaattggctcgagttccaccgctaccgccgcgacatgacgctgatggtcctcgatgtggtctcgctgttctctgccctcgacacgatccgctacccgaacgctacagttgtgcagctcagccgcactgtctacaccgatccgattggcttcgttaaccgcgggtcaggcaataggctgtcctggttcgactggaggaaccaggcgaatttctctactctcgagtcagagatgccgaccccctcatccccactgagcctcaaccacatgtcgatcttcactgggcctctgaccctcccagtgtcccctaacacgcatagggcccgggtctggtacggcaaccagaatatgttcacaactgggtcacagaactccggccagaccacgaactctattcagaatatctcaggcctggagattttccgcatcgactctcaggcgtgcaatctcaataacaattcatacggcgtgaacagggcggagttcttccacggggctagccagggctcgcagcggtctgtctaccagggatacatccgccagagcggcctggacaaccctgtcgttatgaatctgcagtctttcctcccaggcgagaactcagccacccctacggcgcaggattacacccacattctgtccaacccggttaatatcaggggcgggctcaggcagattgtggccgacaggcgctcctccgtggtcgtttacggctggacgcacaagtccctgagcaggaggtcactcgtggctccagaccagatcacccaggtcccagccgttaaggcgtccccttcttcacattgcactatcattgccggcccaggcttcaccggcggggacctggtgtcgctccagcccaacggccagctcgtcatcccgttccaggtttctgcgcccgagacgaactaccacattcgcatctgctacgtctcgacgtctgattgcagcattaacacaatctgcaatgacgagacgcatctgtccacactcccgagcacaacttccagcctggagaacctccagtgcaatcacctgcattacttcaacgtgggcactttcaagccaaccatcgactcgaagctgacgctcgtcaacacatctcctaacgctaacatcattatcgacaagatcgagttcatcccggtggataccgcccagcagcagaacgaggacctcgaggccgcgaagaaggctgtcgcctccctgttcacacgcactagggacggcctccaggtcaatgttaaggactaccaggtggatcaggctgccaacctggtctcatgcctctccgacgagcagtacggctacgataagaagatgctgctcgaggccgtgagggctgctaagaggctgagcagggagaggaacctgctccaggaccccgatttcaacacaatcaactcgaccgaggagaacgggtggaaggcgtcaaatggcgtcaccatctccgagggcgggccattctacaagggcagggctattcagctcgcgtctgctcgggagaactaccccacatacatctaccagaaggtggatgcctccgagctgaagccatacacccgctaccgcctcgacggcttcgtcaagtcgtctcaggacctggagattgatctcatccaccatcacaaggtgcacctggtcaagaacgttccggacaatctcgtgagcatgaacaggaacaacccaaacgagtacgagattattgatgctccatactgcggctgcccctccgatgacgatgtgcgctaccccctcgccagcgacccgaacgccgcgttccagaatatgaactacaaggagtacctgcagacctacgacggcgattacacggggtcactgattaatccaaacctctccatcaatcctcgcgacgtcctccagaccggaatcaacattgttggccgcatcctcggcttcctgggcgtgccgttcgctggccagctggttaccttctacacgttcctcctgaaccagctctggcctacgaatgacaacgcggtgtgggaggccttcatggcgcagatcgaggagctgattgatcagaagatctccgctcaggtggtcaggaacgccctcgacgatctgaccggcctccacgactactacgaggagtacctggctgctctcgaggagtggctcgagaggccaaacggcgctcgcgctaatctggtcacgcagcgcttcgagaacctccataccgccttcgtgacgaggatgccgagcttcgggacaggccccgggtcgcagagggacgcggttgctctcctgactgtgtacgcgcaggcggctaacctgcacctcctgctcctgaaggatgctgagatctacggcgctcggtgggggctgcagcagggccagatcaacctctacttcaatgcccagcaggagcgcacaaggatctacactaaccactgcgttgagacctacaatagggggctcgaggacgtgcggggcacgaacacagagagctggctgaattaccatcgcttccgcagggagatgacgctcatggcgatggacctcgtggcgctcttcccctactacaacgtccgccagtacccaaatggcgccaaccctcagctgacaagggagatctacactgacccgatcgtgtacaacccaccagctaatcaggggatctgcaggcgctggggcaacaatccctacaacaccttctctgagctggagaatgcgttcattaggccacctcacctcttcgaccgcctgaacaggctcaccatctcccggaatcgctacacggctccaaccacgaactcgtacctggattactggtctggccataccctccagtcacagtacgcgaacaatcctacaacttacgagacgtcctacggccagattacaagcaacactcgcctcttcaataccacgaacggcgctaatgctatcgacagcagggcccggaacttcgggaatctgtacgcgaatctctacggcgtctccagcctgaacattttcccaaccggcgttatgtcagagatcacctccgcccctaacacgtgctggcaggacctcacaactaccgaggagctgccactggtgaacaataacttcaatctcctgtcccacgtcacattcctgaggttcaacacgacacagggcggcccactcgcgactgttggcttcgtgcccacctacgtgtggacgcggcaggacgtcgatttcaataacatcattacaccaaaccgcatcactcagattcctgttgtgaaggcgtacgagctgtcgtctggcgctacagtcgttaagggcccggggttcactggcggggacgtcattaggaggactaacaccggcgggttcggggctatcagggtgagcgtcacaggccccctcactcagcgctacaggattcggttccgctacgcgtcgaccatcgacttcgatttcttcgtcacgcgcggcgggactaccatcaataacttccggttcacgcgcaccatgaacaggggccaggagagccggtacgagtcgtaccgcaccgtggagttcacgacaccgttcaacttcacacagagccaggacatcattcgcacttctattcagggcctgtcaggcaacggggaggtttacctcgaccggatcgagatcattccagtgaacccaaccagggaggctgaggaggatctcgaggctgcgaagaaggctgtggcctcgctgttcactaggacccgggacggcctccaggttaatgtgacggactaccaggtggatcaggctgccaacctggtctcgtgcctctctgacgagcagtacgctcacgataagaagatgctcctggaggccgtccgcgctgctaagaggctgtcgagggagaggaacctcctgcaggacccagatttcaacaccattaattctacggaggagaacgggtggaaggcgtcgaatggcgtgaccatctctgagggcgggcctttctacaagggccgcgctctccagctggcttcagctagggagaactacccgacatacatctaccagaaggtcgacgcctccgagctgaagccctacacgcgctaccgcctcgatggcttcgtgaagtcatcccaggacctggagatcgatctcattcaccatcacaaggtccacctggttaagaacgtgctggacaatctcgtcagcgatacctacccggacgattcttgctcaggcatcaatcgctgcgaggagcagcagatggtgaacgcccagctcgagaccgagcatcaccatccgatggactgctgcgaggctgctcagacgcatgagttcagctcgtacatcgacacaggggatctgaactccactgtggaccagggcatctgggtcatcttcaaggtgcgcactaccgatgggtacgcgaccctcggcaacctcgagctggtcgaggttgggccgctcctgggcgagccactggagagggagcagagggagaacgctaagtggaatgctgagctgggcaggaagcgggctgagaccgaccgcgtctaccaggatgctaagcagtccatcaatcacctgttcgtggactaccaggatcagcagctcaacccacagattggcatggctgacatcatggatgcccagaacctggtcgcgtccatcagcgacgtctactctgatgccgttctccagatccctggcattaattacgagatctacacagagctgtcaaaccggctccagcaggcctcctacctgtacactagccgcaacgcggtgcagaatggggacttcaataacggcctcgattcctggaatgctacagctggggctagcgtccagcaggacggcaacactcacttcctcgttctgtctcattgggatgcccaggtttcacagcagttcagggtgcagccgaactgcaagtatgtgctgagggttaccgctgagaaggttggcgggggcgacggctacgtgacgatcagggatggcgctcaccatacggagacactgactttcaacgcctgcgactacgatatcaatggcacctacgtcacggacaacacatacctcactaaggaggtcctcttctacagccacaccgagcatatgtgggtggaggtcaacgagacggagggcgccttccacctcgactcgattgagttcgtggagaccgagaagtga

SEQ ID NO: 15 - DNA, 3468 bp, Artificial Sequence
  Synthetic Cry Gene
atgaataggaataaccaggacgagtacgagatcattgacgcttcgacttgcgggtgcagctcagacgatgttgttcagtaccccctcgctcgcgatcccaatgccgtgttccagaacatgcactacaaggactacctccagacatacgacggcgattacactgggtcgctcattaacccaaatctgtctatcaatcctcgcgacgtcctgcagacgggaatcaacattgttgggaggctcctgggcttcctcggggttccgttcgctggccagctggtgacattctacactttcctcctgaaccagctctggcccaccaacgacaatgcggtctgggaggccttcatggcgcagatcgaggagctgattaaccagcgcatctccgaggctgtggtcggcaccgctgctgatcacctcacggggctgcatgacaactacgagctttacgtggaggctctcgaggagtggctggagaggccaaacgctgctaggacgaacctcctgttcaataggttcaccacgctcgactccctgttcacacagttcatgccatcattcgggactggccccggctcccagaactacgccgtccctctcctgaccgtttacgcgcaggcggctaacctccacctcctgctcctgaaggacgctgagatctacggcgctcgctgggggctgaaccagaatcagatcaacagcttccacacaaggcagcaggagcggacccagtactacacgaatcattgcgtgacaacttacaacaccggcctcgataggctgagggggaccaatacggagtcctggctcaactaccataggttccgcagggagatgaccctgatggcgatggacctcgtggcgctgttcccgtactacaacgtccggcagtacccaaacggcgctaatccacagctcacccgcgagatctacacggacccaatcgtcttcaacccaccagctaatgttggcctgtgcaggcgctgggggaacaatccttacaatcgcttcagcgagctggagaacgccttcatcaggccacctcacctgttcgatcggctcaatacactgactatttcgaggaaccggttcgacgtcggcagcaatttcatcgagccgtggtcgggccatacgctgaggaggtcctacagcaacaattcaacagtgtacgaggattcctacggccagattaccgctacgaggaccacgatcaacctccctgccaatggcacagggcgggtggagtctactgctgtcgacttccgctcagccctggttggcatctacggggtgaacagggcgagcttcatcccgggcggggtcttcagcggcacaactcagccatcgaccggcgggtgcagggacctctacgattccagcgacgagctgccaccagacgagagcacgggctcgttcgctcacaggctctctcatgtcacattcctgtcattcaccacgaaccaggctggctcgatcgccaattctgggagggttccgacatacgtgtggactcaccgggacgtggatttcaacaataccatcaacccaaatcgcatcacgcagattcctgttgtgaaggcgtacgagctgtcctccggcgctaccgtcgttaagggcccggggttcacgggcggggacgtgattcgcaggacaaacatcggcgggttcggcgctatcagggtctccgttaccggccccctgacgcagcgctacaggattcggttccgctacgcctccactatcgacttcgatttcttcgtcacccggggcgggacaactatcaacaatttccgcttcacaaggactatgaacaggggccaggagtcacggtacgagtcctaccgcaccgtggagttcaccacgcccttcaacttcacgcagtcccaggacatcattaggacatccattcagggcctcagcggcaacggggaggtttacctggatcgcatcgagatcattccagtgaaccctacgagggaggctgaggaggacctcgaggctgcgaagaaggctgtggctagcctcttcaccaggacgagggatggcctgcaagtgaatgtcaccgattaccaggtggaccaggctgccaacctcgtctcttgcctgtcagatgagcagtacggccacgacaagaagatgctcctggaggccgtccgcgctgctaagaggctgtccagggagaggaacctcctgcaggacccagatttcaacacaatcaatagcactgaggagaatggctggaaggcgtccaacggggtgaccatcagcgagggcgggcctttctacaagggccgcgctctccagctggcttcggctagggagaattacccaacttacatctaccagaaggtcaacgcctctgagctgaagccttacacgcgctaccgcctggatggcttcgtgaagtcatcccaggatctcgagatcgacctgattcaccatcacaaggtgcacctcgtcaagaacgttccggacaatctggtcagcgatacgtactcggacggctcgtgctctgggatgaatcgctgcgaggagcagcagatggtgaacgcgcagctcgagacagagcatcaccatccgatggactgctgcgaggccgcgcagactcatgagttcagctcgtacattaataccggcgatctgaactcttcagtcgaccagggcatctgggtggtcctcaaggttcgcacaactgatggctacgccacgctggggaacctcgagctggttgaagtgggcccactctccggggagagcctggagagggagcagagggacaacgcgaagtggtccgctgagctgggcaggaagcgggctgagaccgatagggtttaccaggacgctaagcagtccatcaatcacctcttcgtggattaccaggaccagcagctgaacccggagattggcatggctgatatcattgacgcccagaacctcgtcgcgtcaatctccgatgtctacagcgacgccgttctgcagatccccggcattaattacgagatctacacggagctgtcgaacaggctgcagcaggcctcgtacctctacacatctcggaacgcggtgcagaatggcgatttcaactctgggctggactcatggaatgctaccggcggggctacggtgcagcaggatggcaacacccacttcctcgtcctgtcccattgggacgctcaggtgagccagcagttccgggtccagccgaactgcaagtatgtgctgagggtcactgctgagaaggttggcgggggcgatggctacgtgaccatcagggacggggctcaccatacagagaagctcactttcaacgcctgcgactacgatatcaatggcacctacgtcacggacaacacatacatcactaaggaggttgtgttctactcgcacactgagcatatgtgggtcgaggtttctgagaccgagggcgccttccacctcgactcaattgagttcgtggagaccgagaagtga

SEQ ID NO: 16 - protein, 1168 aa, Bacillus thuringiensis
MNRNNQNEYEVIDAPHCGCPADDVVKYPLTDDPNAGLQNMNYKEYLQTYGGDYTDPLINPNLSVSGKDVIQVGINIVGRLLSFFGFPFSSQWVTVYTYLLNSLWPDDENSVWDAFMERVEELIDQKISEAVKGRALDDLTGLQYNYNLYVEALDEWLNRPNGARASLVSQRFNILDSLFTQFMPSFGSGPGSQNYATILLPVYAQAANLHLLLLKDADIYGARWGLNQTQIDQFHSRQQSLTQTYTNHCVTAYNDGLAELRGTSVASWLKYHQYRREMTVTAMDLVALFPYYNVRQYPNGANPQLTREVYTDPIVFNPPERPSGAFCESFYTIRAARERLTFSQLEHAIIRPPRLFERFQALGIYTGEARLNANSAPMNYWIGHFIRNTRLGDSTTITTNYGTTNNRLTNFSMPSDVYQINSTSSNLAAILGTLYGVTRAQFHFGSGSFSTYVGQNSVLPQCHQNYNSIEELPNQSDEPTVRSYSHRLSHITSFNFNVQLNNPLISAGNMPVYVWTHRSVDLTNRISSDRITQIPVVKAYELSSGATVVKGPGFTGGDVIRRTNTGGFGAIRVSVTGPLTQRYRIRFRYASTIDFDFFVTRGGTTINNFRFTRTMNRGQESRYESYRTVEFTTPFNFTQSQDIIRTSIQGLSGNGEVYLDRIEIIPVNPTREAEEDLEAAKKAVASLFTRTRDGLQVNVKDYQVDQAANLVSCLSDEQYGYDKKMLLEAVRAAKRLSRERNLLQDPDFNTINSTEENGWKASNGVTISEGGPFYKGRALQLASARENYPTYIYQKVDASELKPYTRYRLDGFVKSSQDLEIDLIHHHKVHLVKNVPDNLVSDTYPDDSCSGINRCQEQQMVNAQLETEHHHPMDCCEAAQTHEFSSYIDTGDLNSTVDQGIWVIFKVRTTDGYATLGNLELVEVGPLLGEPLEREQRENAKWNAELGRKRAETDRVYQDAKQSINHLFVDYQDQQLNPEIGMADIMDAQNLVASISDVYSDAVLQIPGINYEIYTELSNRLQQASYLYTSRNAVQNGDFNNGLDSWNATAGASVQQDGNTHFLVLSHWDAQVSQQFRVQPNCKYVLRVTAEKVGGGDGYVTIRDDAHHTETLTFNACDYDINGTYVTDNTYLTKEVVFYSHTDHMWVEVSETEGAFHIDSIEFVETEK

SEQ ID NO: 17 - protein, 1156 aa, Bacillus thuringiensis
MNQNKHGIIGASNCGCASDDVAKYPLANNPYSSALNLNSCQNSSILNWINIIGDAAKEAVSIGTTIVSLITAPSLTGLISIVYDLIGKVLGGSSGQSISDLSICDLLSIIDLRVSQSVLNDGIADFNGSVLLYRNYLEALDSWNKNPNSASAEELRTRFRIADSEFDRILTRGSLTNGGSLARQNAQILLLPSFASAAFFHLLLLRDATRYGTNWGLYNATPFINYQSKLVELIELYTDYCVHWYNRGFNELRQRGTSATAWLEFHRYRREMTLMVLDIVASFSSLDITNYPIETDFQLSRVIYTDPIGFVHRSSLRGESWFSFVNRANFSDLENAIPNPRPSWFLNNMIISTGSLTLPVSPSTDRARVWYGSRDRISPANSQFITELISGQHTTATQTILGRNIFRVDSQACNLNDTTYGVNRAVFYHDASEGSQRSVYEGYIRTTGIDNPRVQNINTYLPGENSDIPTPEDYTHILSTTINLTGGLRQVASNRRSSLVMYGWTHKSLARNNTINPDRITQIPLTKVDTRGTGVSYVNDPGFIGGALLQRTDHGSLGVLRVQFPLHLRQQYRIRVRYASTTNIRLSVNGSFGTISQNLPSTMRLGEDLRYGSFAIREFNTSIRPTASPDQIRLTIEPSFIRQEVYVDRIEFIPVNPTREAKEDLEAAKKAVASLFTRTRDGLQVNVKDYQVDQAANLVSCLSDEQYGYDKKMLLEAVRAAKRLSRERNLLQDPDFNTINSTEENGWKASNGVTISEGGPFYKGRAIQLASARENYPTYIYQKVDASELKPYTRYRLDGFVKSSQDLEIDLIHHHKVHLVKNVPDNLVLDTYPDDSCNGINRCDEQKMVNAQLETEHHHPMDCCEAAQTHEFSSYINTGDLNASVDQGIWVVLKVRTTDGYATLGNLELVEVGPLSGESLEREQRDNAKWSAELGRKRAETERVYYAAKQSINHLFVDYRDQQLNPQIGMADIMDAQNLVASISDVYSDAVLQIPGINYEIYTELSNRLQQASYLHMSRNAMQNGDFNSGLDSWNATAGATVQQDGNTHFLVLSHWDAQVSQQFRVQPNCKYVLRVTAEKVGGGDGYVTIRDGAHHTETLTFNACDYDINGTYVTDNTYLTKEVVFHPETQHMWVEVSETEGVFHIDSVEFMETQQ

SEQ ID NO: 18 - protein, 1156 aa, Bacillus thuringiensis
MNQNKHGIIGASNCGCASDDVAKYPLANNPYSSALNLNSCQNSSILNWINIIGDAAKEAVSIGTTIVSLITAPSLTGLISIVYDLIGKVLGGSSGQSISDLSICDLLSIIDLRVSQSVLNDGIADFNGSVLLYRNYLEALDSWNKNPNSASAEELRTRFRIADSEFDRILTRGSLTNGGSLARQNAQILLLPSFASAAFFHLLLLRDATRYGTNWGLYNATPFINYQSKLVELIELYTDYCVHWYNRGFNELRQRGTSATAWLEFHRYRREMTLMVLDIVASFSSLDITNYPIETDFQLSRVIYTDPIGFVHRSSLRGESWFSFVNRANFSDLENAIPNPRPSWFLNNMIISTGSLTLPVSPSTDRARVWYGSRDRISPANSQFITELISGQHTTATQTILGRNIFRVDSQACNLNDTTYGVNRAVFYHDASEGSQRSVYEGYIRTTGIDNPRVQNINTYLPGENSDIPTPEDYTHILSTTINLTGGLRQVASNRRSSLVMYGWTHKSLARNNTINPDRITQIPLTKVDTRGTGVSYVNDPGFIGGALLQRTDHGSLGVLRVQFPLHLRQQYRIRVRYASTTNIRLSVNGSFGTISQNLPSTMRLGEDLRYGSFAIREFNTSIRPTASPDQIRLTIEPSFIRQEVYVDRIEFIPVNPTREAKEDLEAAKKAVASLFTRTRDGLQVNVKDYQVDQAANLVSCLSDEQYGYDKKMLLEAVRAAKRLSRERNLLQDPDFNTINSTEENGWKASNGVTISEGGPFYKGRAIQLASARENYPTYIYQKVDASELKPYTRYRLDGFVKSSQDLEIDLIHHHKVHLVKNVPDNLVLDTYPDDSCNGINRCDEQKMVNAQLETGHHHPMDCCEAAQTHEFSSYINTGDLNASVDQGIWVVLKVRTTDGYATLGNLELVEVGPLSGESLEREQRDNAKWSAELGRKRAETERVYYAAKQSINHLFVDYQDQQLNPQIGMADIMDAQNLVASISDVYSDAVLQIPGINYEIYTELSNRLQQASYLHTSRNAMQNGDFNSGLDSWNATAGATVQQDGNTHFLVLSHWDAQVSQQFRVQPNCKYVLRVTAEKVGGGDGYVTIRDGAHHTETLTFNACDYDINGTYVTDNTYLTKEVVFHPETQHMWVEVSETEGVFHIDSVEFMETQQ

SEQ ID NO: 19 - protein, 1152 aa, Bacillus thuringiensis
MNRNNPNEYEIIDAPYCGCPSDDDVRYPLASDPNAAFQNMNYKEYLQTYDGDYTGSLINPNLSINPRDVLQTGINIVGRILGFLGVPFAGQLVTFYTFLLNQLWPTNDNAVWEAFMAQIEELIDQKISAQVVRNALDDLTGLHDYYEEYLAALEEWLERPNGARANLVTQRFENLHTAFVTRMPSFGTGPGSQRDAVALLTVYAQAANLHLLLLKDAEIYGARWGLQQGQINLYFNAQQERTRIYTNHCVETYNRGLEDVRGTNTESWLNYHRFRREMTLMAMDLVALFPYYNVRQYPNGANPQLTREIYTDPIVYNPPANQGICRRWGNNPYNTFSELENAFIRPPHLFDRLNRLTISRNRYTAPTTNSYLDYWSGHTLQSQYANNPTTYETSYGQITSNTRLFNTTNGANAIDSRARNFGNLYANLYGVSSLNIFPTGVMSEITSAPNTCWQDLTTTEELPLVNNNFNLLSHVTFLRFNTTQGGPLATVGFVPTYVWTRQDVDFNNIITPNRITQIPVVKAYELSSGATVVKGPGFTGGDVIRRTNTGGFGAIRVSVTGPLTQRYRIRFRYASTIDFDFFVTRGGTTINNFRFTRTMNRGQESRYESYRTVEFTTPFNFTQSQDIIRTSIQGLSGNGEVYLDRIEIIPVNPTREAEEDLEAAKKAVASLFTRTRDGLQVNVTDYQVDQAANLVSCLSDEQYAHDKKMLLEAVRAAKRLSRERNLLQDPDFNTINSTEENGWKASNGVTISEGGPFYKGRALQLASARENYPTYIYQKVDASELKPYTRYRLDGFVKSSQDLEIDLIHHHKVHLVKNVLDNLVSDTYPDDSCSGINRCEEQQMVNAQLETEHHHPMDCCEAAQTHEFSSYIDTGDLNSTVDQGIWVIFKVRTTDGYATLGNLELVEVGPLLGEPLEREQRENAKWNAELGRKRAETDRVYQDAKQSINHLFVDYQDQQLNPQIGMADIMDAQNLVASISDVYSDAVLQIPGINYEIYTELSNRLQQASYLYTSRNAVQNGDFNNGLDSWNATAGASVQQDGNTHFLVLSHWDAQVSQQFRVQPNCKYVLRVTAEKVGGGDGYVTIRDGAHHTETLTFNACDYDINGTYVTDNTYLTKEVIFYSHTEHMWVEVNETEGAFHIDSIEFVETEK

SEQ ID NO: 20 - protein, 1155 aa, Bacillus thuringiensis
MNRNNQDEYEIIDASTCGCSSDDVVQYPLARDPNAVFQNMHYKDYLQTYDGDYTGSLINPNLSINPRDVLQTGINIVGRLLGFLGVPFAGQLVTFYTFLLNQLWPTNDNAVWEAFMAQIEELINQRISEAVVGTAADHLTGLHDNYELYVEALEEWLERPNAARTNLLFNRFTTLDSLFTQFMPSFGTGPGSQNYAVPLLTVYAQAANLHLLLLKDAEIYGARWGLNQNQINSFHTRQQERTQYYTNHCVTTYNTGLDRLRGTNTESWLNYHRFRREMTLMAMDLVALFPYYNVRQYPNGANPQLTREIYTDPIVFNPPANVGLCRRWGNNPYNRFSELENAFIRPPHLFDRLNTLTISRNRFDVGSNFIEPWSGHTLRRSYSNNSTVYEDSYGQITATRTTINLPANGTGRVESTAVDFRSALVGIYGVNRASFIPGGVFSGTTQPSTGGCRDLYDSSDELPPDESTGSFAHRLSHVTFLSFTTNQAGSIANSGRVPTYVWTHRDVDFNNTINPNRITQIPVVKAYELSSGATVVKGPGFTGGDVIRRTNIGGFGAIRVSVTGPLTQRYRIRFRYASTIDFDFFVTRGGTTINNFRFTRTMNRGQESRYESYRTVEFTTPFNFTQSQDIIRTSIQGLSGNGEVYLDRIEIIPVNPTREAEEDLEAAKKAVASLFTRTRDGLQVNVTDYQVDQAANLVSCLSDEQYGHDKKMLLEAVRAAKRLSRERNLLQDPDFNTINSTEENGWKASNGVTISEGGPFYKGRALQLASARENYPTYIYQKVNASELKPYTRYRLDGFVKSSQDLEIDLIHHHKVHLVKNVPDNLVSDTYSDGSCSGMNRCEEQQMVNAQLETEHHHPMDCCEAAQTHEFSSYINTGDLNSSVDQGIWVVLKVRTTDGYATLGNLELVEVGPLSGESLEREQRDNAKWSAELGRKRAETDRVYQDAKQSINHLFVDYQDQQLNPEIGMADIIDAQNLVASISDVYSDAVLQIPGINYEIYTELSNRLQQASYLYTSRNAVQNGDFNSGLDSWNATGGATVQQDGNTHFLVLSHWDAQVSQQFRVQPNCKYVLRVTAEKVGGGDGYVTIRDGAHHTEKLTFNACDYDINGTYVTDNTYLTKEVVFYSHTEHMWVEVSETEGAFHIDSIEFVETEK

SEQ ID NO: 21 - protein, 1168 aa, Artificial Sequence
  Mutant BT-0009
MNRNNQNEYEVIDAPHCGCPADDVVKYPLTDDPNAGLQNMNYKEYLQTYGGDYTDPLINPNLSVSGKDVIQVGINIVGRLLSFFGFPFSSQWVTVYTYLLNSLWPDDENSVWDAFMERVEELIDQKISEAVKGRALDDLTGLQYNYNLYVEALDEWLNRPNGARASLVSQRFNILDSLFTQFMPSFGSGPGSQNYATILLPVYAQAANLHLLLLKDADIYGARWGLNQTQIDQFHSRQQSLTQTYTNHCVTAYNDGLAELRGTSVASWLKYHQYRREMTVTAMDLVALFPYYNVRQYPNGANPQLTREVYTDPIVFNPPERPSGAFCESFYTIRAARERLTFSQLEHAIIRPPRLFERFQALGIYTGEARLNANSAPMNYWIGHFIRNTRLGDSTTITTNYGTTNNRLTNFSMPSDVYQINSTSSNLAAILGTLYGVTRAQFHFGSGSFSTYVGQNSVLPQCHQNYNSIEELPNQSDEPTVRSYSHRLSHITSFNFNVQLNNPLISAGNMPVYVWTHRSVDLTNRISSDRITQIPVVKAYELSSGATVVKGPGFTGGDVIRRTNTGGFGAIRVSVTGPLTQRYRIRFRYASTIDFDFFVTRGGTTINNFRFTRTMNRGQESRYESYRTVEFTTPFNFTQSQDIIRTSIQGLSGNGEVYLDRIEIIPVNPTREAEEDLEAAKKAVASLFTRTRDGLQVNVKDYQVDQAANLVSCLSDEQYGYDKKMLLEAVRAAKRLSRERNLLQDPDFNTINSTEENGWKASNGVTISEGGPFYKGRALQLASARENYPTYIYQKVDASELKPYTRYRLDGFVKSSQDLEIDLIHHHKVHLVKNVPDNLVSDTYPDDSCSGINRCQEQQMVNAQLETEHHHPMDCCEAAQTHEFSSYIDTGDLNSTVDQGIWVIFKVRTTDGYATLGNLELVEVGPLLGEPLEREQRENAKWNAELGRKRAETDRVYQDAKQSINHLFVDYQDQQLNPEIGMADIMDAQNLVASISDVYSDAVLQIPGINYEIYTELSNRLQQASYLYTSRNAVQNGDFNNGLDSWNATAGASVQQDGNTHFLVLSHWDAQVSQQFRVQPNCKYVLRVTAEKVGGGDGYVTIRDDAHHTETLTFNACDYDINGTYVTDNTYITKEVVFYSHTDHMWVEVSETEGAFHIDSLEFVETEK

SEQ ID NO: 22 - protein, 1156 aa, Artificial Sequence
  Mutant BT-0012
MNQNKHGIIGASNCGCASDDVAKYPLANNPYSSALNLNSCQNSSILNWINIIGDAAKEAVSIGTTIVSLITAPSLTGLISIVYDLIGKVIGGSSGQSISDLSICDLLSIIDLRVSQSVLNDGIADFNGSVLLYRNYLEALDSWNKNPNSASAEELRTRFRIADSEFDRILTRGSLTNGGSLARQNAQILLLPSFASAAFFHLLLLRDATRYGTNWGLYNATPFINYQSKLVELIELYTDYCVHWYNRGFNELRQRGTSATAWLEFHRYRREMTLMVLDIVASFSSLDITNYPIETDFQLSRVIYTDPIGFVHRSSLRGESWFSFVNRANFSDLENAIPNPRPSWFLNNMIISTGSLTLPVSPSTDRARVWYGSRDRISPANSQFITELISGQHTTATQTILGRNIFRVDSQACNLNDTTYGVNRAVFYHDASEGSQRSVYEGYIRTTGIDNPRVQNINTYLPGENSDIPTPEDYTHILSTTINLTGGLRQVASNRRSSLVMYGWTHKSLARNNTINPDRITQIPLTKVDTRGTGVSYVNDPGFIGGALLQRTDHGSLGVLRVQFPLHLRQQYRIRVRYASTTNIRLSVNGSFGTISQNLPSTMRLGEDLRYGSFAIREFNTSIRPTASPDQIRLTIEPSFIRQEVYVDRIEFIPVNPTREAKEDLEAAKKAVASLFTRTRDGLQVNVKDYQVDQAANLVSCLSDEQYGYDKKMLLEAVRAAKRLSRERNLLQDPDFNTINSTEENGWKASNGVTISEGGPFYKGRAIQLASARENYPTYIYQKVDASELKPYTRYRLDGFVKSSQDLEIDLIHHHKVHLVKNVPDNLVLDTYPDDSCNGINRCDEQKMVNAQLETEHHHPMDCCEAAQTHEFSSYINTGDLNASVDQGIWVVLKVRTTDGYATLGNLELVEVGPLSGESLEREQRDNAKWSAELGRKRAETERVYYAAKQSINHLFVDYRDQQLNPQIGMADIMDAQNLVASISDVYSDAVLQIPGINYEIYTELSNRLQQASYLHMSRNAMQNGDFNSGLDSWNATAGATVQQDGNTHFLVLSHWDAQVSQQFRVQPNCKYVLRVTAEKVGGGDGYVTIRDGAHHTETLTFNACDYDINGTYVTDNTYLTKEVVFHPETQHMWVEVSETEGVFHLDSVEFMETQQ

SEQ ID NO: 23 - protein, 1156 aa, Artificial Sequence
  Mutant BT-0013
MNQNKHGIIGASNCGCASDDVAKYPLANNPYSSALNLNSCQNSSILNWINIIGDAAKEAVSIGTTIVSLITAPSLTGLISIVYDLIGKVIGGSSGQSISDLSICDLLSIIDLRVSQSVLNDGIADFNGSVLLYRNYLEALDSWNKNPNSASAEELRTRFRIADSEFDRILTRGSLTNGGSLARQNAQILLLPSFASAAFFHLLLLRDATRYGTNWGLYNATPFINYQSKLVELIELYTDYCVHWYNRGFNELRQRGTSATAWLEFHRYRREMTLMVLDIVASFSSLDITNYPIETDFQLSRVIYTDPIGFVHRSSLRGESWFSFVNRANFSDLENAIPNPRPSWFLNNMIISTGSLTLPVSPSTDRARVWYGSRDRISPANSQFITELISGQHTTATQTILGRNIFRVDSQACNLNDTTYGVNRAVFYHDASEGSQRSVYEGYIRTTGIDNPRVQNINTYLPGENSDIPTPEDYTHILSTTINLTGGLRQVASNRRSSLVMYGWTHKSLARNNTINPDRITQIPLTKVDTRGTGVSYVNDPGFIGGALLQRTDHGSLGVLRVQFPLHLRQQYRIRVRYASTTNIRLSVNGSFGTISQNLPSTMRLGEDLRYGSFAIREFNTSIRPTASPDQIRLTIEPSFIRQEVYVDRIEFIPVNPTREAKEDLEAAKKAVASLFTRTRDGLQVNVKDYQVDQAANLVSCLSDEQYGYDKKMLLEAVRAAKRLSRERNLLQDPDFNTINSTEENGWKASNGVTISEGGPFYKGRAIQLASARENYPTYIYQKVDASELKPYTRYRLDGFVKSSQDLEIDLIHHHKVHLVKNVPDNLVLDTYPDDSCNGINRCDEQKMVNAQLETGHHHPMDCCEAAQTHEFSSYINTGDLNASVDQGIWVVLKVRTTDGYATLGNLELVEVGPLSGESLEREQRDNAKWSAELGRKRAETERVYYAAKQSINHLFVDYQDQQLNPQIGMADIMDAQNLVASISDVYSDAVLQIPGINYEIYTELSNRLQQASYLHTSRNAMQNGDFNSGLDSWNATAGATVQQDGNTHFLVLSHWDAQVSQQFRVQPNCKYVLRVTAEKVGGGDGYVTIRDGAHHTETLTFNACDYDINGTYVTDNTYLTKEVVFHPETQHMWVEVSETEGVFHLDSVEFMETQQ

SEQ ID NO: 24 - protein, 1152 aa, Artificial Sequence
  Mutant BT-0023
MNRNNPNEYEIIDAPYCGCPSDDDVRYPLASDPNAAFQNMNYKEYLQTYDGDYTGSLINPNLSINPRDVLQTGINIVGRILGFLGVPFAGQLVTFYTFLLNQLWPTNDNAVWEAFMAQIEELIDQKISAQVVRNALDDLTGLHDYYEEYLAALEEWLERPNGARANLVTQRFENLHTAFVTRMPSFGTGPGSQRDAVALLTVYAQAANLHLLLLKDAEIYGARWGLQQGQINLYFNAQQERTRIYTNHCVETYNRGLEDVRGTNTESWLNYHRFRREMTLMAMDLVALFPYYNVRQYPNGANPQLTREIYTDPIVYNPPANQGICRRWGNNPYNTFSELENAFIRPPHLFDRLNRLTISRNRYTAPTTNSYLDYWSGHTLQSQYANNPTTYETSYGQITSNTRLFNTTNGANAIDSRARNFGNLYANLYGVSSLNIFPTGVMSEITSAPNTCWQDLTTTEELPLVNNNFNLLSHVTFLRFNTTQGGPLATVGFVPTYVWTRQDVDFNNIITPNRITQIPVVKAYELSSGATVVKGPGFTGGDVIRRTNTGGFGAIRVSVTGPLTQRYRIRFRYASTIDFDFFVTRGGTTINNFRFTRTMNRGQESRYESYRTVEFTTPFNFTQSQDIIRTSIQGLSGNGEVYLDRIEIIPVNPTREAEEDLEAAKKAVASLFTRTRDGLQVNVTDYQVDQAANLVSCLSDEQYAHDKKMLLEAVRAAKRLSRERNLLQDPDFNTINSTEENGWKASNGVTISEGGPFYKGRALQLASARENYPTYIYQKVDASELKPYTRYRLDGFVKSSQDLEIDLIHHHKVHLVKNVLDNLVSDTYPDDSCSGINRCEEQQMVNAQLETEHHHPMDCCEAAQTHEFSSYIDTGDLNSTVDQGIWVIFKVRTTDGYATLGNLELVEVGPLLGEPLEREQRENAKWNAELGRKRAETDRVYQDAKQSINHLFVDYQDQQLNPQIGMADIMDAQNLVASISDVYSDAVLQIPGINYEIYTELSNRLQQASYLYTSRNAVQNGDFNNGLDSWNATAGASVQQDGNTHFLVLSHWDAQVSQQFRVQPNCKYVLRVTAEKVGGGDGYVTIRDGAHHTETLTFNACDYDINGTYVTDNTYLTKEVLFYSHTEHMWVEVNETEGAFHLDSIEFVETEK

SEQ ID NO: 25 - protein, 1155 aa, Artificial Sequence
  Mutant BT-0067
MNRNNQDEYEIIDASTCGCSSDDVVQYPLARDPNAVFQNMHYKDYLQTYDGDYTGSLINPNLSINPRDVLQTGINIVGRLLGFLGVPFAGQLVTFYTFLLNQLWPTNDNAVWEAFMAQIEELINQRISEAVVGTAADHLTGLHDNYELYVEALEEWLERPNAARTNLLFNRFTTLDSLFTQFMPSFGTGPGSQNYAVPLLTVYAQAANLHLLLLKDAEIYGARWGLNQNQINSFHTRQQERTQYYTNHCVTTYNTGLDRLRGTNTESWLNYHRFRREMTLMAMDLVALFPYYNVRQYPNGANPQLTREIYTDPIVFNPPANVGLCRRWGNNPYNRFSELENAFIRPPHLFDRLNTLTISRNRFDVGSNFIEPWSGHTLRRSYSNNSTVYEDSYGQITATRTTINLPANGTGRVESTAVDFRSALVGIYGVNRASFIPGGVFSGTTQPSTGGCRDLYDSSDELPPDESTGSFAHRLSHVTFLSFTTNQAGSIANSGRVPTYVWTHRDVDFNNTINPNRITQIPVVKAYELSSGATVVKGPGFTGGDVIRRTNIGGFGAIRVSVTGPLTQRYRIRFRYASTIDFDFFVTRGGTTINNFRFTRTMNRGQESRYESYRTVEFTTPFNFTQSQDIIRTSIQGLSGNGEVYLDRIEIIPVNPTREAEEDLEAAKKAVASLFTRTRDGLQVNVTDYQVDQAANLVSCLSDEQYGHDKKMLLEAVRAAKRLSRERNLLQDPDFNTINSTEENGWKASNGVTISEGGPFYKGRALQLASARENYPTYIYQKVNASELKPYTRYRLDGFVKSSQDLEIDLIHHHKVHLVKNVPDNLVSDTYSDGSCSGMNRCEEQQMVNAQLETEHHHPMDCCEAAQTHEFSSYINTGDLNSSVDQGIWVVLKVRTTDGYATLGNLELVEVGPLSGESLEREQRDNAKWSAELGRKRAETDRVYQDAKQSINHLFVDYQDQQLNPEIGMADIIDAQNLVASISDVYSDAVLQIPGINYEIYTELSNRLQQASYLYTSRNAVQNGDFNSGLDSWNATGGATVQQDGNTHFLVLSHWDAQVSQQFRVQPNCKYVLRVTAEKVGGGDGYVTIRDGAHHTEKLTFNACDYDINGTYVTDNTYITKEVVFYSHTEHMWVEVSETEGAFHLDSIEFVETEK

SEQ ID NO: 26 - DNA, 26 bp, Artificial Sequence
  OAR2613a Forward Primer
aaacatgaaccgaaataatcaaaatg

SEQ ID NO: 27 - DNA, 22 bp, Artificial Sequence
  OAR2615a Reverse Primer
atccgtcccttgtgcgtgtaaa

SEQ ID NO: 28 - DNA, 30 bp, Artificial Sequence
  OAR2611a-F forward primer
gtttaaacatgaatcgaaataatcaaaatg

SEQ ID NO: 29 - DNA, 29 bp, Artificial Sequence
  OAR2612a-R reverse primer
ggcgcgccctactcttgtgtttcaataaa

SEQ ID NO: 30 - DNA, 29 bp, Artificial Sequence
  OAR2768-F forward primer
gtttaaacatgaatcaaaataaacacgga

SEQ ID NO: 31 - DNA, 31 bp, Artificial Sequence
  OAR2769-R reverse primer
ggcgcgccttactgttgggtttccatgaact